European Patent Application EP 4 549 466 A1, published May 7, 2025. Title: 一种新型多特异肿瘤抑制剂的开发和应用. Applicant: 康诺亚生物医药科技（成都）有限公司. The sequence listing filed with the application follows.

SEQUENCE LISTING (275 sequences)

SEQ ID NO: 1 - protein, 345 aa, Homo sapiens
MYKDCIESTGDYFLLCDAEGPWGIILESLAILGIVVTILLLLAFLFLMRKIQDCSQWNVLPTQLLFLLSVLGLFGLAFAFIIELNQQTAPVRYFLFGVLFALCFSCLLAHASNLVKLVRGCVSFSWTTILCIAIGCSLLQIIIATEYVTLIMTRGMMFVNMTPCQLNVDFVVLLVYVLFLMALTFFVSKATFCGPCENWKQHGRLIFITVLFSIIIWVVWISMLLRGNPQFQRQPQWDDPVVCIALVTNAWVFLLLYIVPELCILYRSCRQECPLQGNACPVTAYQHSFQVENQELSRARDSDGAEEDVALTSYGTPIQPQTVDPTQECFIPQAKLSPQQDAGGV

SEQ ID NO: 2 - protein, 344 aa, Macaca fascicularis
MYKDCIESTGDYFLPCDSEGPWGIVLESLAILGIVVTILLLLAFLFLMRKIQDCSQWNVLPTQLLFLLSVLGLFGLAFAFIIQLNQQTAPVRYFLFGVLFALCFSCLLAHASNLVKLVRGRVSFSWTTILCIAIGCSLLQVIIAIEYVTLIMTRGMMFVHMTPYQLNVDFVVLLVYVLFLMALTFFVSKATFCGPCENWKQHGRLIFITVLFSIIIWVVWISMLLRGNPQFQRQPQWDDPVVCIALVTNAWVFLLLYIVPELCILYRSCRQECPSQGHACPVTAYQRSFQVENQELSRARDSDGAEEDVALTSFGTPIQPQTVDPTQECFIPRAKLSPQQDAGV

SEQ ID NO: 3 - protein, 120 aa, synthetic construct
QAYLQQSGAELVRSGASVKMSCKASGYTFTSYNMHWVKQTPGQGLEWIGYIYPGNGGTNYNQKFKAKATLTADTSSSTAYMQISSLTSEDSAVYFCARGYGYRYWYFDVWGAGTTVTVSS

SEQ ID NO: 4 - DNA, 360 bp, synthetic construct
  source 1..360: mol_type = other DNA
caggcttatctacagcagtctggggctgagctggtgaggtctggggcctcagtgaagatgtcctgcaaggcttctggctacacatttaccagttacaatatgcactgggtaaagcagacacctgggcagggcctggaatggattggatatatttatcctggaaatggtggtactaactacaatcagaagttcaaggccaaggccacattgactgcagacacatcctccagcacagcctacatgcagatcagcagcctgacatctgaagactctgcggtctatttctgtgcaagagggtatggttaccgctactggtacttcgatgtctggggcgcagggaccacggtcaccgtctcctca

SEQ ID NO: 5 - protein, 6 aa, synthetic construct
TSYNMH

SEQ ID NO: 6 - protein, 17 aa, synthetic construct
YIYPGNGGTNYNQKFKA

SEQ ID NO: 7 - protein, 11 aa, synthetic construct
GYGYRYWYFDV

SEQ ID NO: 8 - protein, 106 aa, synthetic construct
NIVLTQSPAIMSASPGEKVTMTCSASSSVRFMHWYQQKSGTSPKRWIYDTSKVASGVPARFSGSGSGTSYSLTIRSMEAEDAATYYCQQWSSNPLTFGAGTKLELK

SEQ ID NO: 9 - DNA, 318 bp, synthetic construct
  source 1..318: mol_type = other DNA
aatattgtgctaactcagtctccagcaatcatgtctgcatctccaggggagaaggtcaccatgacctgcagtgccagctcaagtgtacgtttcatgcactggtaccagcagaagtcaggcacctcccccaaaagatggatttatgatacatccaaagtggcttctggagtccctgctcgcttcagtggcagtgggtctgggacctcttactctctcacaatcagaagcatggaggctgaagatgctgccacttattactgccagcagtggagtagtaacccgctcacgttcggtgctgggaccaagctggagctgaaa

SEQ ID NO: 10 - protein, 10 aa, synthetic construct
SASSSVRFMH

SEQ ID NO: 11 - protein, 7 aa, synthetic construct
DTSKVAS

SEQ ID NO: 12 - protein, 9 aa, synthetic construct
QQWSSNPLT

SEQ ID NO: 13 - protein, 113 aa, synthetic construct
QVQLQQPGAELVKPGASVKLSCKASGYTFTRYWMHWVKQRPGQGLDWIGEFNPSNGRINYNEKFKNKATLTIDKSSSTAYMQLSSLTSEDSAVYYCTRGFAYWGQGTLVTVSA

SEQ ID NO: 14 - DNA, 339 bp, synthetic construct
  source 1..339: mol_type = other DNA
caggtccaactgcagcagcctggggctgaactggtgaagcctggggcttcagtgaagctgtcctgcaaggcttctggctacaccttcacccgctactggatgcactgggtgaagcagaggcctggacaaggccttgattggattggagagtttaatcctagtaacggtcgtattaactacaatgagaagttcaagaacaaggccacactgactatagacaagtcctccagcactgcctacatgcaactcagcagcctgacatctgaggactctgcggtctattactgtacaagagggtttgcttactggggccaagggactctggtcactgtctctgca

SEQ ID NO: 15 - protein, 6 aa, synthetic construct
TRYWMH

SEQ ID NO: 16 - protein, 17 aa, synthetic construct
EFNPSNGRINYNEKFKN

SEQ ID NO: 17 - protein, 4 aa, synthetic construct
GFAY

SEQ ID NO: 18 - protein, 106 aa, synthetic construct
QIVLTQSPAIMSASPGERVTMTCSASSTVSYIHWYQQKSGTSPKRWIYDTSKLASGVPARFSGSGSGTSYSLTISSMEAEDAATYYCQQWTTNPWTFGGGTKLEIK

SEQ ID NO: 19 - DNA, 318 bp, synthetic construct
  source 1..318: mol_type = other DNA
caaattgttctcacccagtctccagcaatcatgtctgcatctccaggggagagggtcaccatgacctgcagtgccagctcaactgtaagttacatacactggtaccagcagaagtcaggcacctcccccaaaagatggatttatgacacatccaaactggcttctggagtccctgctcgcttcagtggcagtgggtctgggacctcttactctctcacaatcagcagcatggaggctgaagatgctgccacttattactgccagcagtggactactaacccgtggacgttcggtggaggcaccaagctggaaatcaaa

SEQ ID NO: 20 - protein, 10 aa, synthetic construct
SASSTVSYIH

SEQ ID NO: 21 - protein, 7 aa, synthetic construct
DTSKLAS

SEQ ID NO: 22 - protein, 9 aa, synthetic construct
QQWTTNPWT

SEQ ID NO: 23 - protein, 118 aa, synthetic construct
EVLLQQSGPELVKPGTSMKISCKASGYSFTGYTMNWVKQRHGKNLEWIGLINPYNGGTRYNQKFKGRATLTVDKSSSTAYMELLSLTSEDSAVYYCARWALRYGMDYWGQGTSVTVSS

SEQ ID NO: 24 - DNA, 354 bp, synthetic construct
  source 1..354: mol_type = other DNA
gaggtcctgctgcaacagtctggacctgaactggtgaagcctggaacttcaatgaagatatcctgcaaggcttctggttactcattcactggctacaccatgaactgggtgaaacagagacatggaaagaaccttgagtggattggacttatcaatccttacaatggtggtactaggtacaaccagaagttcaagggcagggccacattaactgtggacaagtcatccagcacagcctacatggaactcctcagtctgacatctgaggactctgcagtctattactgtgcaagatgggccctacggtatggtatggactactggggtcaaggaacctcagtcaccgtctcctca

SEQ ID NO: 25 - protein, 6 aa, synthetic construct
TGYTMN

SEQ ID NO: 26 - protein, 17 aa, synthetic construct
LINPYNGGTRYNQKFKG

SEQ ID NO: 27 - protein, 9 aa, synthetic construct
WALRYGMDY

SEQ ID NO: 28 - protein, 107 aa, synthetic construct
DIVMTQSQKFMSTSVGDRVSVTCKASQNVGTNVAWYQQKPGHSPKALIYSASYRNSGVPDRFTGSGSGTDFTLTISNVQSEDLAEYFCQQYNSYLLTFGGGTKLELK

SEQ ID NO: 29 - DNA, 321 bp, synthetic construct
  source 1..321: mol_type = other DNA
gacattgtgatgacccagtctcaaaaattcatgtccacatcagtaggagacagggtcagcgtcacctgcaaggccagtcagaacgtgggtactaatgtagcctggtatcaacagaaaccagggcattctcctaaagcactgatttactcggcatcctaccggaatagtggagtccctgatcgcttcacaggcagtggctctgggacagatttcactctcaccatcagcaatgtgcagtctgaagacttggcagagtatttctgtcagcaatataacagctatcttctcacgttcggaggggggaccaagctggagctgaaa

SEQ ID NO: 30 - protein, 11 aa, synthetic construct
KASQNVGTNVA

SEQ ID NO: 31 - protein, 7 aa, synthetic construct
SASYRNS

SEQ ID NO: 32 - protein, 9 aa, synthetic construct
QQYNSYLLT

SEQ ID NO: 33 - protein, 120 aa, synthetic construct
QAYLQQSGAELVRSGASVKMSCKASGYTFTSYNMHWVKQTPGQGLEWIGYIYPGNGGTNYNQNFKGKATLTADTSSSTAYMQISSLTSEDSAVYFCARGYGYRYWYFDVWGAGTTVTVSS

SEQ ID NO: 34 - DNA, 360 bp, synthetic construct
  source 1..360: mol_type = other DNA
caggcttatctacagcagtctggggctgagctggtgaggtctggggcctcagtgaagatgtcctgtaaggcttctggctacacatttaccagttacaatatgcactgggtaaagcagacacctggacagggcctggaatggattggatatatttatcctggaaatggtggtactaactacaatcagaatttcaagggcaaggccacattgactgcagacacttcctccagcacagcctacatgcagatcagcagtctgacatctgaagactctgcggtctatttctgtgcaagagggtatggttaccgctactggtacttcgatgtctggggcgcagggaccacggtcaccgtctcctca

SEQ ID NO: 35 - protein, 17 aa, synthetic construct
YIYPGNGGTNYNQNFKG

SEQ ID NO: 36 - protein, 106 aa, synthetic construct
QIVLTQSPAIMSASPGEKVTMTCSASSSVSYMHWYQQKSGTSPKRWIYDTSKLASGVPVRFSGSGSGTSYSLTISSMEAEDAATYYCQQWSNYPPTFGSGTKLEIK

SEQ ID NO: 37 - DNA, 318 bp, synthetic construct
  source 1..318: mol_type = other DNA
caaattgttctcacccagtctccagcaatcatgtctgcatctccaggggagaaggtcaccatgacctgcagtgccagctcaagtgtaagttacatgcactggtaccagcagaagtcaggcacctcccccaaaagatggatttatgacacatccaaactggcttctggagtccctgttcgtttcagtggcagtgggtctgggacctcttactctctcacaatcagcagcatggaggctgaagatgctgccacttattactgccagcagtggagtaattacccacccacgttcggctcggggacaaagttggaaataaaa

SEQ ID NO: 38 - protein, 10 aa, synthetic construct
SASSSVSYMH

SEQ ID NO: 39 - protein, 9 aa, synthetic construct
QQWSNYPPT

SEQ ID NO: 40 - protein, 114 aa, synthetic construct
QVQLQQSGAELVKPGASVKMSCKAFGYTFTNFPIEWMKQNRGRSLEWIGNFHPYNDVTKYNEKFKGKAKLTVEKSSSTVYLELSRLTSDDSAVYYCALITRGYWGQGTTLTVSS

SEQ ID NO: 41 - DNA, 342 bp, synthetic construct
  source 1..342: mol_type = other DNA
caggttcagctgcaacagtctggggctgagctggtgaagcctggggcctcagtgaagatgtcctgcaaggcttttggctacaccttcactaactttccaatagagtggatgaagcagaatcgtgggaggagcctagagtggattggaaattttcatccttacaatgatgttactaagtacaatgaaaaattcaagggcaaggccaaattgactgtagagaaatcctctagcacagtctacttggagctcagccgattaacatctgatgactctgctgtttattactgtgcccttattacacggggctactggggccaaggcaccactctcacagtctcctca

SEQ ID NO: 42 - protein, 6 aa, synthetic construct
TNFPIE

SEQ ID NO: 43 - protein, 17 aa, synthetic construct
NFHPYNDVTKYNEKFKG

SEQ ID NO: 44 - protein, 5 aa, synthetic construct
ITRGY

SEQ ID NO: 45 - protein, 113 aa, synthetic construct
DIVMSQSPSSLGVSVGEKVTMSCKSSQSLLYSRNQKNSLAWYQQKPGQSPKLLIYWASTRESGVPDRFTGSGSGTDFTLTISSVKAEDLAVYYCQQYYSYPLTFGAGTKLELK

SEQ ID NO: 46 - DNA, 339 bp, synthetic construct
  source 1..339: mol_type = other DNA
gacattgtgatgtcacagtctccatcctccctaggtgtgtcagttggagagaaggttactatgagctgcaagtccagtcagagccttttatatagtcgcaatcaaaagaactccttggcctggtaccagcagaaacctgggcagtctcctaaactgctgatttactgggcatccactagggaatctggggtccctgatcgcttcacaggcagtggatctgggacagatttcactctcaccatcagcagtgtgaaggctgaagacctggcagtttattactgtcagcaatattatagctatccgctcacgttcggtgctgggaccaagctggagctgaaa

SEQ ID NO: 47 - protein, 17 aa, synthetic construct
KSSQSLLYSRNQKNSLA

SEQ ID NO: 48 - protein, 7 aa, synthetic construct
WASTRES

SEQ ID NO: 49 - protein, 9 aa
QQYYSYPLT

SEQ ID NO: 50 - protein, 120 aa, synthetic construct
QAYLQQSGAELVRSGASVKMSCKASGYTFTSYNMHWVKQTPGQGLEWIGYIYPGNGGTNYNQKFKGKATLTADTSSSTAYMQISSLTSEDSAVYFCARGYGYRYWYFDVWGTGTTVTVSS

SEQ ID NO: 51 - DNA, 360 bp, synthetic construct
  source 1..360: mol_type = other DNA
caggcttatctacagcagtctggggctgagctggtgaggtctggggcctcagtgaagatgtcctgcaaggcttctggctacacatttaccagttataatatgcactgggtaaagcagacacctgggcagggcctggaatggattggatatatttatcctggaaatggtggtactaactacaatcagaaattcaagggcaaggccacattgactgcagacacatcctccagcacagcctacatgcagatcagcagcctgacatctgaagactctgcggtctatttctgtgcaagagggtatggttaccgctactggtacttcgatgtctggggcacagggaccacggtcaccgtctcctca

SEQ ID NO: 52 - protein, 17 aa, synthetic construct
YIYPGNGGTNYNQKFKG

SEQ ID NO: 53 - protein, 106 aa, synthetic construct
QIVLTQSPAIMSASPGEKVTMTCSASSSVSYMHWYQQKSGTSPKRWIYDTSKLASGVPARFSGSGSGTSYSLTISSMEAEDAATYYCQQWNSKPPTFGSGTKLEIK

SEQ ID NO: 54 - DNA, 318 bp, synthetic construct
  source 1..318: mol_type = other DNA
caaattgttctcacccagtctccagcaatcatgtctgcatctccaggggagaaggtcaccatgacctgcagtgccagctcaagtgtaagttacatgcactggtaccagcagaagtcaggcacctcccccaaaagatggatttatgacacatccaaactggcttctggagtccctgctcgcttcagtggcagtgggtctgggacctcatactctctcacaatcagcagcatggaggctgaagatgctgccacttattactgccaacagtggaatagtaagccacccacgttcggctcggggacaaagttggaaataaaa

SEQ ID NO: 55 - protein, 9 aa, synthetic construct
QQWNSKPPT

SEQ ID NO: 56 - protein, 120 aa, synthetic construct
EVQLVESGGDLVKPGGSLKLSCAASGFTFSSYGMSWVRQTPDKRLEWVATISSGGSYTYYPDSVKGRFTISRDNAKNTLYLQMSSLKSEDTAMYYCARHGGSSSYVMDYWGQGTSVTVSS

SEQ ID NO: 57 - DNA, 360 bp, synthetic construct
  source 1..360: mol_type = other DNA
gaggtgcagctggtggagtctgggggagacttagtgaagcctggagggtccctgaaactctcctgtgcagcctctggattcactttcagtagctatggcatgtcttgggttcgccagactccagacaagaggctggagtgggtcgcaaccattagtagtggtggtagttacacctactatccagacagtgtgaaggggcgattcaccatctccagggacaatgccaagaacaccctgtacctgcaaatgagcagtctgaagtctgaggacacagccatgtattactgtgcaagacatgggggtagtagctcttatgttatggactactggggtcaaggaacctcagtcaccgtctcctca

SEQ ID NO: 58 - protein, 6 aa, synthetic construct
SSYGMS

SEQ ID NO: 59 - protein, 17 aa, synthetic construct
TISSGGSYTYYPDSVKG

SEQ ID NO: 60 - protein, 11 aa, synthetic construct
HGGSSSYVMDY

SEQ ID NO: 61 - protein, 112 aa, synthetic construct
DIVMTQAAPSVPVTPGESVSISCRSSKSLLHSNGNTYLYWFLQRPGQSPQLLIYRMSNLASGVPDRFSGSGSGTAFTLRISRVEAEDVGVYYCMQHLEYPFTFGSGTKLEIK

SEQ ID NO: 62 - DNA, 336 bp, synthetic construct
  source 1..336: mol_type = other DNA
gatattgtgatgactcaggctgcaccctctgtacctgtcactcctggagagtcagtatccatctcctgcaggtctagtaagagtctcctgcatagtaatggcaacacttacttgtattggttcctgcagaggccaggccagtctcctcagctcctgatatatcggatgtccaaccttgcctcaggagtcccagacaggttcagtggcagtgggtcaggaactgctttcacactgagaatcagtagagtggaggctgaggatgtgggtgtttattactgtatgcaacatctagaatatcctttcacgttcggctcggggacaaagttggaaataaaa

SEQ ID NO: 63 - protein, 16 aa, synthetic construct
RSSKSLLHSNGNTYLY

SEQ ID NO: 64 - protein, 7 aa, synthetic construct
RMSNLAS

SEQ ID NO: 65 - protein, 9 aa, synthetic construct
MQHLEYPFT

SEQ ID NO: 66 - protein, 121 aa, synthetic construct
QVQLQQPGAELVKPGASVKLSCKASGYTFTSYYMYWVKQRPGQGLEWIGGINPSNGGTKYNEKFKSKATLTVDKSSSTAFMQLSSLTSEDSAVYYCTRGSLRSYYYAMDYWGQGTSVTVSS

SEQ ID NO: 67 - DNA, 363 bp, synthetic construct
  source 1..363: mol_type = other DNA
caggtccaactgcagcagcctggggctgaactggtgaagcctggggcttcagtgaagttgtcctgcaaggcttctggctacaccttcaccagctattatatgtactgggtgaagcagaggcctggacaaggccttgagtggattggggggattaatcctagcaatggtggtactaagtacaatgagaagttcaagagcaaggccacactgactgtagacaaatcctccagcacagccttcatgcaactcagcagcctgacatctgaggactctgcggtctattactgtacaagaggatcactacggtcttattactatgctatggactactggggtcaaggaacctcagtcaccgtctcctca

SEQ ID NO: 68 - protein, 6 aa, synthetic construct
TSYYMY

SEQ ID NO: 69 - protein, 17 aa, synthetic construct
GINPSNGGTKYNEKFKS

SEQ ID NO: 70 - protein, 12 aa, synthetic construct
GSLRSYYYAMDY

SEQ ID NO: 71 - protein, 107 aa, synthetic construct
DIQMTQTTSSLSASLGDRVTISCRASQDISNYLNWYQQKPDGTVKLLIYYTSRLHSGVPSRFSGSGSGTDYSLTISNLEQEDLATYFCQQGYSLPYTFGGGTKLEIK

SEQ ID NO: 72 - DNA, 321 bp, synthetic construct
  source 1..321: mol_type = other DNA
gatatccagatgacacagactacatcctccctgtctgcctctctgggagacagagtcaccatcagttgcagggcaagtcaggacattagtaattatttaaactggtatcagcagaaaccagatggaactgttaaactcctgatctactacacatcaagattacattcaggagtcccatcaaggttcagtggcagtgggtctggaacagattattctctcaccattagcaacctggagcaagaagatcttgccacttatttttgccaacagggttattcgcttccgtacacgttcggaggggggaccaagctggaaataaaa

SEQ ID NO: 73 - protein, 11 aa, synthetic construct
RASQDISNYLN

SEQ ID NO: 74 - protein, 7 aa, synthetic construct
YTSRLHS

SEQ ID NO: 75 - protein, 9 aa, synthetic construct
QQGYSLPYT

SEQ ID NO: 76 - protein, 123 aa, synthetic construct
QVQLQQSGAELARPGASVKMSCKASGYIFTSYTMYWVKQRPGQGLEWIGYINPSSGYTNYNQKFKDKATLTADKSSSTAYMQLSSLTSEDSAVYYCARWGGNERLYYYAMDYWGQGTSVTVSS

SEQ ID NO: 77 - DNA, 369 bp, synthetic construct
  source 1..369: mol_type = other DNA
caggtccagctgcagcagtctggggctgaactggcaagacctggggcctcagtgaagatgtcctgcaaggcttctggctacatctttactagctacacgatgtactgggtaaaacagaggcctggacagggtctggaatggattggatacattaatcctagcagtggttatactaattacaatcagaagttcaaggacaaggccacattgactgcagacaaatcctccagcacagcctacatgcaactgagcagcctgacatctgaggactctgcagtctattactgtgcaagatggggtggtaacgaacgcctatattactatgctatggactactggggtcaaggaacctcagtcaccgtctcctca

SEQ ID NO: 78 - protein, 17 aa, synthetic construct
YINPSSGYTNYNQKFKD

SEQ ID NO: 79 - protein, 14 aa, synthetic construct
WGGNERLYYYAMDY

SEQ ID NO: 80 - protein, 106 aa, synthetic construct
QIVLTQSPAIMSASPGEKVTITCSASSSVSYMYWFQQKPGTSPKLWIYGTSNLASGVPARFSGSGSGTSYSLTISRMEAEDAATYYCQQRSSYPLTFGAGTKLELK

SEQ ID NO: 81 - DNA, 318 bp, synthetic construct
  source 1..318: mol_type = other DNA
caaattgttctcacccagtctccagcaatcatgtctgcatctccaggggagaaggtcaccataacctgcagtgccagctcaagtgtaagttacatgtactggttccagcagaagccaggcacttctcccaaactctggatttatggcacatccaacctggcttctggagtccctgctcgcttcagtggcagtggatctgggacctcttactctctcacaatcagccgaatggaggctgaagatgctgccacttattactgccagcagaggagcagttacccgctcacgttcggtgctgggaccaagctggagctgaaa

SEQ ID NO: 82 - protein, 10 aa, synthetic construct
SASSSVSYMY

SEQ ID NO: 83 - protein, 7 aa, synthetic construct
GTSNLAS

SEQ ID NO: 84 - protein, 9 aa, synthetic construct
QQRSSYPLT

SEQ ID NO: 85 - protein, 113 aa, synthetic construct
DIVMSQSPSSLAVSVGEKVTMSCKSSQSLLYSRNQKNSLAWYQQKPGQSPKLLLYWASTRESGVPDRFTGSGSGTDFTLTISSVKAEDLAVYYCQQYYSYPLTFGAGTKLELK

SEQ ID NO: 86 - DNA, 339 bp, synthetic construct
  source 1..339: mol_type = other DNA
gacattgtgatgtcacagtctccatcctccctagctgtgtcagttggagagaaggttactatgagctgcaagtccagtcagagccttttatatagtcgcaatcaaaagaactccttggcctggtaccagcagaaacctgggcagtctcctaaactgctgctttactgggcatccactagggaatctggggtccctgatcgcttcacaggcagtggatctgggacagatttcactctcaccatcagcagtgtgaaggctgaagacctggcagtttattactgtcagcaatattatagctatccgctcacgttcggtgctgggaccaagctggagctgaaa

SEQ ID NO: 87 - protein, 118 aa, synthetic construct
EVQLQQSGPELVKPGASMKISCKASGYSFTGYTMNWVKQRHGKNLEWIGLINPYNGGTSYNQKFKGKATLTVDKSSSTAYMELLSLTSEDSAVYYCARLPIRNGMDYWGQGTSVTVSS

SEQ ID NO: 88 - DNA, 354 bp, synthetic construct
  source 1..354: mol_type = other DNA
gaggtccagctgcagcagtctggacctgagctggtgaagcctggagcttcaatgaagatatcctgcaaggcttctggttactcattcactggctacaccatgaactgggtgaagcagaggcatggaaagaaccttgagtggattggacttattaatccttacaatggaggtactagctataaccagaagttcaagggcaaggccacattaactgtagacaagtcatccagcacagcctacatggagctcctcagtctgacatctgaggactctgcagtctattactgtgcaagattacctatccgaaatggtatggactactggggtcaaggaacctcagtcaccgtctcctca

SEQ ID NO: 89 - protein, 17 aa, synthetic construct
LINPYNGGTSYNQKFKG

SEQ ID NO: 90 - protein, 9 aa, synthetic construct
LPIRNGMDY

SEQ ID NO: 91 - protein, 107 aa, synthetic construct
DIVLTQSPATLSVTPGDSVSLSCRASQSISNNLHWYQQKSHESPRLLVKFASLSISGIPSRFSGSGSGTDFTLSINSVETEDFGMYFCQQSNSWPQTFGGGTKLEIK

SEQ ID NO: 92 - DNA, 321 bp, synthetic construct
  source 1..321: mol_type = other DNA
gatattgtgctaactcagtctccagccaccctgtctgtgactccaggagatagcgtcagtctttcctgcagggccagccaaagtattagcaacaacctacactggtatcaacaaaaatcacatgagtctccaaggcttctcgtcaaatttgcttccctgtccatctctgggatcccctccaggttcagtggcagtggatcagggacagatttcactctcagtatcaacagtgtggagactgaagattttggaatgtatttctgtcaacagagtaacagctggcctcagacgttcggtggaggcaccaagctggaaatcaaa

SEQ ID NO: 93 - protein, 11 aa, synthetic construct
RASQSISNNLH

SEQ ID NO: 94 - protein, 7 aa, synthetic construct
FASLSIS

SEQ ID NO: 95 - protein, 9 aa, synthetic construct
QQSNSWPQT

SEQ ID NO: 96 - protein, 121 aa, synthetic construct
EVQLQQSGPELVKPGASVKMSCKASEYTFTNYVMYWVKQKPGQGLEWIGYINPYNDGTKYNEKFKGKATLTSDKSSSTAYMELSSLTSEDSAVYYCVRGGMLTTRSLFTYWGQGTLVTVSA

SEQ ID NO: 97 - DNA, 363 bp, synthetic construct
  source 1..363: mol_type = other DNA
gaggtccagctgcagcagtctggacctgagctggtaaagcctggggcttcagtgaagatgtcctgcaaggcttctgaatacacattcactaattatgttatgtattgggtgaagcagaagcctgggcagggccttgagtggattggatatattaatccttacaatgatggtactaagtacaatgagaagttcaaaggcaaggccacactgacttcagacaaatcctccagcacagcctacatggagctcagcagcctgacctctgaggactctgcggtctattactgtgtgagagggggaatgcttacgacgcgttccctttttacttactggggccaagggactctggtcactgtctctgca

SEQ ID NO: 98 - protein, 6 aa, synthetic construct
TNYVMY

SEQ ID NO: 99 - protein, 17 aa, synthetic construct
YINPYNDGTKYNEKFKG

SEQ ID NO: 100 - protein, 12 aa, synthetic construct
GGMLTTRSLFTY

SEQ ID NO: 101 - protein, 107 aa, synthetic construct
DIQMTQSPSSLSASLGERVSLTCRASQRISGYLSWLQQKPDGTIKRLIYAASTLDSGVPKRFSGSRSGSDYSLTISSLESEDFADYYCLQYASYPPTFGGGTKLEIK

SEQ ID NO: 102 - DNA, 321 bp, synthetic construct
  source 1..321: mol_type = other DNA
gacatccagatgacccagtctccatcctccttatctgcctctctgggagaaagagtcagtctcacttgtcgggcaagtcaaagaattagtggttacttaagctggcttcagcaaaaaccagatggaactattaaacgcctgatctacgccgcatccactttagattctggtgtcccaaaaaggttcagtggcagtaggtctgggtcagattattctctcaccatcagcagccttgagtctgaagattttgcagactattactgtctacaatatgctagttatcctccgacgttcggtggaggcaccaagctggaaatcaaa

SEQ ID NO: 103 - protein, 11 aa, synthetic construct
RASQRISGYLS

SEQ ID NO: 104 - protein, 7 aa, synthetic construct
AASTLDS

SEQ ID NO: 105 - protein, 9 aa, synthetic construct
LQYASYPPT

SEQ ID NO: 106 - protein, 121 aa, synthetic construct
EVQLQQSGPDLVKPGASVKMSCKASGYKFTSYVMYWVKQKTGQGLEWIGYINPYNDGTKYNEKFKGKATLTSDKSSSTAYMEFSSLTSEDSAVYYCVRGGMLTTRSLFAYWGQGTLVTVSA

SEQ ID NO: 107 - DNA, 363 bp, synthetic construct
  source 1..363: mol_type = other DNA
gaggtccagctgcagcagtctggacctgacctggtaaagcctggggcttcagtgaagatgtcctgcaaggcttctggatacaaattcactagctatgttatgtactgggtgaagcagaagactgggcagggccttgagtggattggatatattaatccttacaatgatggtactaagtacaatgagaagttcaaaggcaaggccacactgacttcagacaaatcctccagcacagcctacatggagttcagcagcctgacctctgaggactctgcggtctattactgtgtaagagggggaatgcttacgacgcgttccctttttgcttactggggccaagggactctggtcactgtctctgca

SEQ ID NO: 108 - protein, 6 aa, synthetic construct
TSYVMY

SEQ ID NO: 109 - protein, 12 aa, synthetic construct
GGMLTTRSLFAY

SEQ ID NO: 110 - protein, 107 aa, synthetic construct
DIQMTQSPSSLSASLGERVSLTCRASQEISGYFSWLQQKPDGTIKRLIYAASTLDSGVPKRFSGSRSGSDYSLTISSLESEDFADYYCLQYASYPPTFGGGTKLEIK

SEQ ID NO: 111 - DNA, 321 bp, synthetic construct
  source 1..321: mol_type = other DNA
gacatccagatgacccagtctccatcctccttatctgcctctctgggagaaagagtcagtctcacttgtcgggcaagtcaggaaattagtggttactttagctggcttcagcagaaaccagatggaactattaaacgcctgatctacgccgcatccactttagattctggtgtcccaaaaaggttcagtggcagtaggtctgggtcagattattctctcaccatcagcagccttgagtctgaagattttgcagactattactgtctacaatatgctagttatcctccgacgttcggtggaggcaccaagctggaaatcaaa

SEQ ID NO: 112 - protein, 11 aa, synthetic construct
RASQEISGYFS

SEQ ID NO: 113 - protein, 121 aa, synthetic construct
EVQLQQSGPELVKPGASVKMSCKASGYTFTNYVMYWVKQKPGQVLEWIGYINPYNDGTKYNEKFTGKATLTSDKSSSTAYMELSSLTSEDSAVYYCARGGMLTTRSLFVYWGQGTLVTVSA

SEQ ID NO: 114 - DNA, 363 bp, synthetic construct
  source 1..363: mol_type = other DNA
gaggtccagctgcagcagtctggacctgagctggtaaagcctggggcttcagtgaagatgtcctgcaaggcttctggatacacattcactaactatgttatgtactgggtgaaacagaagcctgggcaggtccttgaatggattggatatattaatccttacaatgatggtactaagtacaatgagaagttcacaggcaaggccacactgacttcagacaaatcctccagcacagcctacatggagctcagcagcctgacctctgaggactctgcggtctattactgtgcaagagggggaatgcttacgacgcgttccctttttgtttactggggccaagggactctggtcactgtctctgca

SEQ ID NO: 115 - protein, 17 aa, synthetic construct
YINPYNDGTKYNEKFTG

SEQ ID NO: 116 - protein, 12 aa, synthetic construct
GGMLTTRSLFVY

SEQ ID NO: 117 - protein, 118 aa, synthetic construct
EVQLQQSGPELGKPGASVKMSCKASGYTFTNYVMHWVKQKPGQGLEWIGYINPYNDGTKYNEKFKGKATLTSDKSSNTAYMELSSLTSEDSAVYYCARGGVRRYFDYWGQGTTLTVSS

SEQ ID NO: 118 - DNA, 354 bp, synthetic construct
  source 1..354: mol_type = other DNA
gaggtccagctgcagcagtctggacctgagctgggaaagcctggggcttcagtgaagatgtcctgcaaggcttctggatacacattcactaactatgttatgcactgggtgaagcagaagcctgggcagggccttgagtggattggatatattaatccttacaatgatggtactaagtacaatgagaagttcaaaggcaaggccacactgacttcagacaaatcctccaacacagcctacatggagctcagcagcctgacctctgaggactctgcggtctattactgtgcaagaggaggggtacgacgctactttgactactggggccaaggcaccactctcacagtctcctca

SEQ ID NO: 119 - protein, 6 aa, synthetic construct
TNYVMH

SEQ ID NO: 120 - protein, 9 aa, synthetic construct
GGVRRYFDY

SEQ ID NO: 121 - protein, 107 aa, synthetic construct
DIQMTQSPSSLSASLGERVSLTCRASQDIGSNLNWLQQEPDGTIKRLIYATSSLDSGVPKRFSGSRSGSDYSLTISSLESEDFVDYYCLQYASFPYTFGGGTKLEIK

SEQ ID NO: 122 - DNA, 321 bp, synthetic construct
  source 1..321: mol_type = other DNA
gacatccagatgacccagtctccatcctccttatctgcctctctgggagaaagagtcagtctcacttgtcgggcaagtcaggacattggtagtaacttaaactggcttcagcaggaaccagatggaactattaaacgcctgatctacgccacatccagtttagattctggtgtccccaaaaggttcagtggcagtaggtctgggtcagattattctctcaccatcagcagccttgagtctgaagattttgtagactattactgtctacaatatgctagttttccgtacacgttcggaggggggaccaagctggaaataaaa

SEQ ID NO: 123 - protein, 11 aa, synthetic construct
RASQDIGSNLN

SEQ ID NO: 124 - protein, 7 aa, synthetic construct
ATSSLDS

SEQ ID NO: 125 - protein, 9 aa, synthetic construct
LQYASFPYT

SEQ ID NO: 126 - protein, 121 aa, synthetic construct
EVQLQQSGPELVKPGASVKMSCMASGYTFTSYVMYWVKQKPGQGLEWIGYINPYNDGTKYNEKFKGKATLTSDKSSSTAYMELSSLTSEDSAVYYCARGGMLTTRSLFVYWGHGTLVTVSA

SEQ ID NO: 127 - DNA, 363 bp, synthetic construct
  source 1..363: mol_type = other DNA
gaggtccagctgcagcagtctggacctgaactggtaaagcctggggcttcagtgaagatgtcctgcatggcttctggatacacattcactagctatgttatgtactgggtgaagcagaagcctgggcagggccttgagtggattggatatattaatccttacaatgatggtactaagtacaatgagaagttcaaaggcaaggccacactgacttcagacaaatcctccagcacagcctacatggagctcagcagcctgacctctgaggactctgcggtctattactgtgcaagagggggaatgcttacgacgcgttccctttttgtttactggggccacgggactctggtcactgtctctgca

SEQ ID NO: 128 - protein, 107 aa, synthetic construct
DIQMTQSPSSLSASLGERVSLTCRASQEISGYLSWLQQKPDGTIKRLIYAASTLDSGVPKRFSGSRSGSDYSLTISSLESEDFADYYCLQYASYPPTYGGGTKLEIK

SEQ ID NO: 129 - DNA, 321 bp, synthetic construct
  source 1..321: mol_type = other DNA
gacatccagatgacccagtctccatcctccttatctgcctctctgggagaaagagtcagtctcacttgtcgggcaagtcaggaaattagtggttacttaagctggcttcagcagaaaccagatggaactattaaacgcctgatctacgccgcatccactttagattctggtgtcccaaaaaggttcagtggcagtaggtctgggtcagattattctctcaccatcagcagccttgagtctgaagattttgcagactattactgtctacaatatgctagttatcctccgacgtacggtggaggcaccaagctggaaatcaaa

SEQ ID NO: 130 - protein, 11 aa, synthetic construct
RASQEISGYLS

SEQ ID NO: 131 - protein, 121 aa, synthetic construct
EVQLQQSGPELVKPGASVKMSCKASGYTFTSYVMYWVKQKPGQVLEWIGYINPYNDGTKYNERFTGKATLTSDKSSSTAYMELSSLTSEDSAVYYCARGGMLTTRSLFLYWGQGTLVTVSA

SEQ ID NO: 132 - DNA, 363 bp, synthetic construct
  source 1..363: mol_type = other DNA
gaggtccagctgcagcagtctggacctgagctggtaaagcctggggcttcagtgaagatgtcctgcaaggcttctggatacacattcactagttatgttatgtactgggtgaaacagaagcctgggcaggtccttgaatggattggatatattaatccttacaatgatggtactaagtacaatgagaggttcacaggcaaggccacactgacttcagacaaatcctccagcacagcctacatggagctcagcagcctgacctctgaggactctgcggtctattactgtgcaagagggggaatgcttacgacgcgttccctttttctttactggggccaagggactctggtcactgtctctgca

SEQ ID NO: 133 - protein, 17 aa, synthetic construct
YINPYNDGTKYNERFTG

SEQ ID NO: 134 - protein, 12 aa, synthetic construct
GGMLTTRSLFLY

SEQ ID NO: 135 - protein, 107 aa, synthetic construct
DIVMSQSPSSLSASLGERVSLTCRASQEISGYFSWLQQKPDGTIKRLIYAASTLDSGVPKRFSGSRSGSDYSLTISSLESEDFADYYCLQYASYPPTFGGGTKLEIK

SEQ ID NO: 136 - DNA, 321 bp, synthetic construct
  source 1..321: mol_type = other DNA
gacattgtgatgtcacagtctccatcctccttatctgcctctctgggagaaagagtcagtctcacttgtcgggcaagtcaggaaattagtggttactttagctggcttcagcagaaaccagatggaactattaaacgcctgatctacgccgcatccactttagattctggtgtcccaaaaaggttcagtggcagtaggtctgggtcagattattctctcaccatcagcagccttgagtctgaagattttgcagactattactgtctacaatatgctagttatcctccgacgttcggtggaggcaccaagctggaaataaaa

SEQ ID NO: 137 - protein, 118 aa, synthetic construct
EVQLVESGGDLVKPGGSLKLSCAASGFTFSSYGMSWVRQTPDKRLEWVATISSGGSYTYYPDSVKGRFTISRDNAKNTLYLQMSSLKSEDTAMYYCARHEARATFDYWGQGTTLTVSS

SEQ ID NO: 138 - DNA, 354 bp, synthetic construct
  source 1..354: mol_type = other DNA
gaggtgcagctggtggagtctgggggagacttagtgaagcctggagggtccctgaaactctcctgtgcagcctctggattcactttcagtagctatggcatgtcttgggttcgccagactccagacaagaggctggagtgggtcgcaaccattagtagtggtggtagttacacctactatccagacagtgtgaaggggcgattcaccatctccagagacaatgccaagaacaccctgtacctgcaaatgagcagtctgaagtctgaggacacagccatgtattactgtgcaagacatgaggctcgggctacctttgactactggggccaaggcaccactctcacagtctcctca

SEQ ID NO: 139 - protein, 9 aa, synthetic construct
HEARATFDY

SEQ ID NO: 140 - protein, 121 aa, synthetic construct
EVQLQQSGPELVKPGASVKMSCKASEYTFTNYVMYWVKQKPGQGLEWIGYINPYNDGTKYNEKFKGKATLTSDKSSSTAYMELSSLTSEDSAVYYCVRGGMLTTRSLFAYWGQGTLVTVSA

SEQ ID NO: 141 - DNA, 363 bp, synthetic construct
  source 1..363: mol_type = other DNA
gaggtccagctgcagcagtctggacctgagctggtaaagcctggggcttcagtgaagatgtcctgcaaggcttctgaatacacattcactaattatgttatgtattgggtgaagcagaagcctgggcagggccttgagtggattggatatattaatccttacaatgatggtactaagtacaatgagaagttcaaaggcaaggccacactgacttcagacaaatcctccagcacagcctacatggagctcagcagcctgacctctgaggactctgcggtctattactgtgtgagagggggaatgcttacgacgcgttccctttttgcttactggggccaagggactctggtcactgtctctgca

SEQ ID NO: 142 - protein, 107 aa, synthetic construct
DIQMTQSPSSLSASLGERVSLTCRASQRISGYLSWLQQKPDGTIKRLIYAASTLDSGVPKRFSGSRSGSDYSLTISSLESEDFADYYCLQYANYPPTFGGGTKLEIK

SEQ ID NO: 143 - DNA, 321 bp, synthetic construct
  source 1..321: mol_type = other DNA
gacatccagatgacccagtctccatcctccttatctgcctctctgggagaaagagtcagtctcacttgtcgggcaagtcaaagaattagtggttacttaagctggcttcagcaaaaaccagatggaactattaaacgcctgatctacgccgcatccactttagattctggtgtcccaaaaaggttcagcggcagtaggtctgggtcagattattctctcaccatcagcagccttgagtctgaagattttgcagactattactgtctacaatatgctaattatcctccgacgttcggtggaggcaccaagctggaaatcaaa

SEQ ID NO: 144 - protein, 9 aa, synthetic construct
LQYANYPPT

SEQ ID NO: 145 - protein, 118 aa, synthetic construct
EVQLQQSGPELVKPGTSMKISCKASGYSFTGYTMNWVKQSHGKNLEWIGLINPYNGGSNYNLKFKGKATLTVDKSSNTAYMELLSLTSEDSAVYYCARWGLRNAMDYWGQGTSVTVSS

SEQ ID NO: 146 - DNA, 354 bp, synthetic construct
  source 1..354: mol_type = other DNA
gaggtccagctgcagcagtctggacctgagctggtgaagcctggaacttcaatgaagatatcctgcaaggcttctggttactcattcactggctacaccatgaactgggtgaagcagagccatggaaagaaccttgagtggattggacttattaatccttacaatggtggttctaactacaacctgaagttcaagggcaaggccacattaactgtagacaagtcatccaacacagcctacatggaactcctcagtctgacatctgaggactctgcagtctattactgtgcaagatggggattacggaatgctatggactactggggtcaaggaacctcagtcaccgtctcctca

SEQ ID NO: 147 - protein, 17 aa, synthetic construct
LINPYNGGSNYNLKFKG

SEQ ID NO: 148 - protein, 9 aa, synthetic construct
WGLRNAMDY

SEQ ID NO: 149 - protein, 107 aa, synthetic construct
DIVVTQSPATLSVTPGDSVSLSCRASQSISNNLHWFQQKSHESPRLLIKYASQSISGIPSRFSGSGSGTDFTLSINSVETEDFGMYFCQQSNSWPQTFGGGTKLEIK

SEQ ID NO: 150 - DNA, 321 bp, synthetic construct
  source 1..321: mol_type = other DNA
gatattgtggtaactcagtctccagccaccctgtctgtgactccaggagatagcgtcagtctttcctgcagggccagtcaaagtattagcaacaacctacactggtttcaacaaaaatcacatgagtctccaaggcttctcatcaagtatgcttcccagtccatctctgggatcccctccaggttcagtggcagtggatcagggacagatttcactctcagtatcaacagtgtggagactgaagattttggaatgtatttctgtcaacagagtaacagttggcctcagacgttcggtggaggcaccaagctggaaatcaaa

SEQ ID NO: 151 - protein, 7 aa, synthetic construct
YASQSIS

SEQ ID NO: 152 - protein, 109 aa, synthetic construct
QAVVTQEPSLTVSPGGTVTLTCRSSTGAVTTSNYANWVQEKPGQAPRGLIGGTNKRAPWTPARFSGSLLGGKAALTITGAQAEDEAEYYCVLWYSNLWVFGGGTKLTVL

SEQ ID NO: 153 - DNA, 327 bp, synthetic construct
  source 1..327: mol_type = other DNA
caggctgtggtcacacaagagcctagcctgacagtgtctcctggcggcacagtgaccctgacctgtagatcttctacaggcgccgtgaccaccagcaactacgctaattgggtgcaggagaagcccggccaggctcctagaggactgatcggcggaacaaacaagagagccccttggacacccgccagattctctggatctctgctcggcggaaaggccgctctgacaatcactggtgctcaggctgaggacgaggccgagtactattgtgtgctgtggtacagcaacctgtgggtgttcggcggaggcaccaaactgacagttctg

SEQ ID NO: 154 - protein, 14 aa, synthetic construct
RSSTGAVTTSNYAN

SEQ ID NO: 155 - protein, 8 aa, synthetic construct
GGTNKRAP

SEQ ID NO: 156 - protein, 9 aa, synthetic construct
VLWYSNLWV

SEQ ID NO: 157 - protein, 125 aa, synthetic construct
EVQLVESGGGLVQPGGSLRLSCAASGFTFNTYAMNWVRKAPGKGLEWVGRIRSKYNNYATYYADSVKDRFTISRDDSKNSLYLQMNSLKTEDTAVYYCVRHGNFGNSYVSWFAYWGQGTLVTVSS

SEQ ID NO: 158 - DNA, 375 bp, synthetic construct
  source 1..375: mol_type = other DNA
gaggtgcagctggttgaatctggcggaggactggttcagcctggcggatctctgagactgtcttgtgccgccagcggcttcaccttcaacacctacgctatgaactgggtccgaaaggcccctggcaaaggactggaatgggtgggaagaatcaggtccaagtacaacaactacgccacctactacgccgacagcgtgaaggacagattcaccatcagcagggacgacagcaagaacagcctgtacctgcagatgaacagcctgaaaaccgaggacaccgccgtgtactactgtgtcagacacggcaacttcggcaacagctatgtgtcttggtttgcctactggggccagggcacactggtcacagttagctct

SEQ ID NO: 159 - protein, 6 aa, synthetic construct
NTYAMN

SEQ ID NO: 160 - protein, 18 aa, synthetic construct
IRSKYNNYATYYADSVKD

SEQ ID NO: 161 - protein, 14 aa, synthetic construct
HGNFGNSYVSWFAY

SEQ ID NO: 162 - protein, 113 aa, synthetic construct
QVQLVQSGAEVKKPGSSVKVSCKASGYTFTRYWMHWVREAPGQGLEWMGEFNPSNGRINYNEKFQGRVTLTIDKSSSTAYMELSSLRSEDTAVYYCTRGFAYWGQGTLVTVSS

SEQ ID NO: 163 - DNA, 339 bp, synthetic construct
  source 1..339: mol_type = other DNA
caggttcagctggttcagtctggcgccgaagtgaagaaacctggcagcagcgtgaaggtgtcctgcaaggctagcggctacacattcaccagatactggatgcactgggtccgagaggcccctggacaaggacttgagtggatgggcgagttcaaccccagcaacggcagaatcaactacaacgagaagttccagggcagagtgaccctgaccatcgacaagagcagcagcaccgcctacatggaactgagcagcctgagaagcgaggacaccgccgtgtactactgcacaagaggcttcgcttactggggccagggaaccctggttaccgttagctct

SEQ ID NO: 164 - protein, 17 aa, synthetic construct
EFNPSNGRINYNEKFQG

SEQ ID NO: 165 - protein, 106 aa, synthetic construct
EIVLTQSPATLSLSPGERATLSCRASSTVSYIHWYQKKPGQAPRRLIYDTSKLASGIPARFSGSGSGTDYTLTISSLEPEDFAVYYCQQWTTNPWTFGGGTKVEIK

SEQ ID NO: 166 - DNA, 318 bp, synthetic construct
  source 1..318: mol_type = other DNA
gagatcgtgctgacacagagccctgccacactgtcactgtctccaggcgagagagccacactgagctgtagagccagcagcaccgtgtcctacatccactggtatcagaagaagcccggccaggctcctagaaggctgatctacgacacaagcaagctggcctctggcatccccgctagattttctggcagcggcagcggaaccgactacaccctgacaatcagcagcctggaacctgaggacttcgccgtgtactactgccagcagtggaccaccaatccttggacattcggcggaggcaccaaggtggaaatcaag

SEQ ID NO: 167 - protein, 10 aa, synthetic construct
RASSTVSYIH

SEQ ID NO: 168 - protein, 118 aa, synthetic construct
QVQLVQSGAEVKKPGSSVKVSCKASGYSFTGYTMNWVREAPGQGLEWMGLINPYNGGTRYNQKFQGRVTLTVDKSSSTAYMELSSLRSEDTAVYYCARWALRYGMDYWGQGTLVTVSS

SEQ ID NO: 169 - DNA, 354 bp, synthetic construct
  source 1..354: mol_type = other DNA
caggttcagctggttcagtctggcgccgaagtgaagaaacctggcagcagcgtgaaggtgtcctgcaaggctagcggctacagcttcaccggctacaccatgaactgggtccgagaggctcctggacagggactcgaatggatgggcctgatcaacccttacaacggcggcaccagatacaaccagaaattccagggcagagtgaccctgaccgtggacaagtctagcagcaccgcctacatggaactgagcagcctgagaagcgaggacaccgccgtgtactactgtgccagatgggctctgagatacggcatggactactggggccagggaaccctggttaccgttagctct

SEQ ID NO: 170 - protein, 17 aa, synthetic construct
LINPYNGGTRYNQKFQG

SEQ ID NO: 171 - protein, 107 aa, synthetic construct
DIQMTQSPSSLSASVGDRVTITCRASQNVGTNVAWYQKKPGKAPKALIYSASYRNSGVPSRFSGSGSGTDFTLTISSLQPEDFATYFCQQYNSYLLTFGGGTKVEIK

SEQ ID NO: 172 - DNA, 321 bp, synthetic construct
  source 1..321: mol_type = other DNA
gacatccagatgacacagagccctagcagcctgtctgccagcgtgggagacagagtgaccatcacctgtagagccagccagaacgtgggcacaaacgtggcctggtatcagaagaagcctggcaaggcccctaaggctctgatctacagcgccagctacagaaacagcggcgtgccctctagattcagcggctctggctctggcaccgacttcaccctgacaatctctagcctgcagcctgaggacttcgctacctacttctgccagcagtacaacagctacctgctgaccttcggcggaggcaccaaggtggaaatcaag

SEQ ID NO: 173 - protein, 11 aa, synthetic construct
RASQNVGTNVA

SEQ ID NO: 174 - protein, 120 aa, synthetic construct
QAQLVQSGAEVKKPGSSVKVSCKASGYTFTSYNMHWVREAPGQGLEWMGYIYPGNGGTNYNQKFQGRVTLTADTSSSTAYMELSSLRSEDTAVYFCARGYGYRYWYFDVWGQGTLVTVSS

SEQ ID NO: 175 - DNA, 360 bp, synthetic construct
  source 1..360: mol_type = other DNA
caggctcagctggttcagtctggcgccgaagtgaagaaacctggcagcagcgtgaaggtgtcctgcaaggctagcggctacacattcaccagctacaacatgcactgggtccgagaggcccctggacagggacttgagtggatgggctacatctaccctggcaacggcggcaccaactacaaccagaaattccagggcagagtgaccctgaccgccgacacatctagcagcaccgcctacatggaactgagcagcctgagaagcgaggataccgccgtgtacttctgtgccagaggctacggataccggtactggtacttcgacgtgtggggccagggaaccctggtcacagtttcttct

SEQ ID NO: 176 - protein, 17 aa, synthetic construct
YIYPGNGGTNYNQKFQG

SEQ ID NO: 177 - protein, 106 aa, synthetic construct
EIVLTQSPATLSLSPGERATLSCRASSSVSYMHWYQKKPGQAPRRLIYDTSKLASGIPARFSGSGSGTDYTLTISSLEPEDFAVYYCQQWSNYPPTFGGGTKVEIK

SEQ ID NO: 178 - DNA, 318 bp, synthetic construct
  source 1..318: mol_type = other DNA
gagatcgtgctgacacagagccctgccacactgtcactgtctccaggcgagagagccacactgagctgtagagccagcagcagcgtgtcctacatgcactggtatcagaagaagcccggccaggctcctagaaggctgatctacgacacaagcaagctggcctctggcatccccgctagattttctggcagcggcagcggaaccgactacaccctgacaatcagcagcctggaacctgaggacttcgccgtgtactactgccagcagtggtctaactaccctcctaccttcggcggaggcaccaaggtggaaatcaag

SEQ ID NO: 179 - protein, 10 aa, synthetic construct
RASSSVSYMH

SEQ ID NO: 180 - protein, 114 aa, synthetic construct
QVQLVQSGAEVKKPGSSVKVSCKASGYTFTNFPIEWMREAPGQGLEWMGNFHPYNDVTKYNEKFQGRVTLTVDKSSSTVYMELSSLRSEDTAVYYCALITRGYWGQGTLVTVSS

SEQ ID NO: 181 - DNA, 342 bp, synthetic construct
  source 1..342: mol_type = other DNA
caggttcagctggttcagtctggcgccgaagtgaagaaacctggcagcagcgtgaaggtgtcctgcaaggctagcggctacacattcacaaacttccccatcgagtggatgagagaggcccctggacagggccttgagtggatgggaaactttcacccctacaacgacgtgaccaagtacaacgagaagttccagggcagagtgaccctgaccgtggacaagagcagcagcaccgtgtacatggaactgagcagcctgagaagcgaggacaccgccgtgtactactgtgccctgatcaccagaggctactggggccagggaacactggtcacagtcagctct

SEQ ID NO: 182 - protein, 17 aa, synthetic construct
NFHPYNDVTKYNEKFQG

SEQ ID NO: 183 - protein, 113 aa, synthetic construct
DIVMTQSPDSLAVSLGERATINCKSSQSLLYSRNQKNSLAWYQKKPGQPPKLLIYWASTRESGVPDRFSGSGSGTDFTLTISSLQAEDVAVYYCQQYYSYPLTFGQGTKLEIK

SEQ ID NO: 184 - DNA, 339 bp, synthetic construct
  source 1..339: mol_type = other DNA
gacatcgtgatgacacagagccctgatagcctggccgtgtctctgggagagagagccaccatcaactgcaagagcagccagagcctgctgtactccagaaaccagaagaacagcctggcctggtatcagaagaagcccggccagcctcctaagctgctgatctactgggccagcaccagagaaagcggcgtgccagatagattcagcggcagcggctctggaaccgacttcaccctgacaatcagctccctgcaggccgaggatgtggccgtgtactactgccagcagtactacagctaccctctgaccttcggccagggcaccaagctggaaatcaag

SEQ ID NO: 185 - protein, 121 aa, synthetic construct
QVQLVQSGAEVKKPGSSVKVSCKASGYTFTSYYMYWVREAPGQGLEWMGGINPSNGGTKYNEKFQGRVTLTVDKSSSTAYMELSSLRSEDTAVYYCTRGSLRSYYYAMDYWGQGTLVTVSS

SEQ ID NO: 186 - DNA, 363 bp, synthetic construct
  source 1..363: mol_type = other DNA
caggttcagctggttcagtctggcgccgaagtgaagaaacctggcagcagcgtgaaggtgtcctgcaaggctagcggctacacattcaccagctactacatgtactgggtccgagaggctcctggacagggactcgaatggatgggcggcatcaacccttctaacggcggcaccaagtacaacgagaagttccagggcagagtgaccctgaccgtggacaagtctagcagcaccgcctacatggaactgagcagcctgagaagcgaggacaccgccgtgtactactgtaccagaggctccctgagatcctactactacgccatggactactggggccagggcacactggttaccgttagctct

SEQ ID NO: 187 - protein, 17 aa, synthetic construct
GINPSNGGTKYNEKFQG

SEQ ID NO: 188 - protein, 107 aa, synthetic construct
DIQMTQSPSSLSASVGDRVTITCQASQDISNYLNWYQKKPGKAPKLLIYYTSRLHSGVPSRFSGSGSGTDYTFTISSLQPEDIATYFCQQGYSLPYTFGQGTKLEIK

SEQ ID NO: 189 - DNA, 321 bp, synthetic construct
  source 1..321: mol_type = other DNA
gacatccagatgacacagagccctagcagcctgtctgccagcgtgggagacagagtgaccatcacctgtcaggccagccaggacatcagcaactacctgaactggtatcagaagaagcccggcaaggcccctaagctgctgatctactacaccagcagactgcacagcggcgtgccctctagattttctggcagcggctctggcaccgactacaccttcacaatcagcagcctgcagcctgaggatatcgctacctacttctgccagcaaggctacagcctgccttacacattcggccagggcaccaagctggaaatcaag

SEQ ID NO: 190 - protein, 11 aa, synthetic construct
QASQDISNYLN

SEQ ID NO: 191 - protein, 118 aa, synthetic construct
QVQLVQSGAEVKKPGSSVKVSCKASGYTFTNYVMHWVKEKPGQGLEWMGYINPYNDGTKYNEKFQGRVTLTSDKSSNTAYMELSSLRSEDTAVYYCARGGVRRYFDYWGQGTLVTVSS

SEQ ID NO: 192 - DNA, 354 bp, synthetic construct
  source 1..354: mol_type = other DNA
caggttcagctggttcagtctggcgccgaagtgaagaaacctggcagcagcgtgaaggtgtcctgcaaggctagcggctacacattcaccaactacgtgatgcactgggtcaaagagaagcccggccagggacttgagtggatgggctacatcaacccctacaacgacggcaccaagtacaacgagaagttccagggcagagtgaccctgaccagcgacaagtctagcaacaccgcctacatggaactgagcagcctgagaagcgaggacaccgccgtgtactactgtgctagaggcggagtgcggagatacttcgactactggggacagggcaccctggtcacagtctcttct

SEQ ID NO: 193 - protein, 17 aa, synthetic construct
YINPYNDGTKYNEKFQG

SEQ ID NO: 194 - protein, 107 aa, synthetic construct
DIQMTQSPSSLSASVGDRVTITCRASQDIGSNLNWLQKEPGKAPKRLIYATSSLDSGVPSRFSGSRSGSDYTLTISSLQPEDFATYYCLQYASFPYTFGQGTKLEIK

SEQ ID NO: 195 - DNA, 321 bp, synthetic construct
  source 1..321: mol_type = other DNA
gacatccagatgacacagagccctagcagcctgtctgccagcgtgggagacagagtgaccatcacctgtagagccagccaggacatcggcagcaacctgaactggctgcagaaagagcctggcaaggcccctaagagactgatctacgccacaagcagcctggacagcggagtgccttctagattcagcggcagcagaagcggcagcgactacaccctgacaatcagcagtctgcagcccgaggacttcgccacctactactgtctgcagtacgctagcttcccctacaccttcggccagggcaccaagctggaaatcaag

SEQ ID NO: 196 - protein, 445 aa, synthetic construct
QVQLVQSGAEVKKPGSSVKVSCKASGYSFTGYTMNWVREAPGQGLEWMGLINPYNGGTRYNQKFQGRVTLTVDKSSSTAYMELSSLRSEDTAVYYCARWALRYGMDYWGQGTLVTVSSASTKGPSVFPLAPCSRSTSESTAALGCLVKDYFPEPVTVSWNSGALTSGVHTFPAVLQSSGLYSLSSVVTVPSSSLGTKTYTCNVDHKPSNTKVDKRVESKYGPPCPPCPAPEFEGGPSVFLFPPKPKDTLMISRTPEVTCVVVDVSQEDPEVQFNWYVDGVEVHNAKTKPREEQFNSTYRVVSVLTVLHQDWLNGKEYKCKVSNKGLASSIEKTISKAKGQPREPQVCTLPPSQEEMTKNQVSLSCAVKGFYPSDIAVEWESNGQPENNYKTTPPVLDSDGSFFLVSKLTVDKSRWQEGNVFSCSVMHEALHNHYTQKSLSLSLGK

SEQ ID NO: 197 - DNA, 1335 bp, synthetic construct
  source 1..1335: mol_type = other DNA
caggttcagctggttcagtctggcgccgaagtgaagaaacctggcagcagcgtgaaggtgtcctgcaaggctagcggctacagcttcaccggctacaccatgaactgggtccgagaggctcctggacagggactcgaatggatgggcctgatcaacccttacaacggcggcaccagatacaaccagaaattccagggcagagtgaccctgaccgtggacaagtctagcagcaccgcctacatggaactgagcagcctgagaagcgaggacaccgccgtgtactactgtgccagatgggctctgagatacggcatggactactggggccagggaaccctggttaccgttagctctgctagcaccaagggccccagcgtgttccccctggccccttgcagcagaagcaccagcgagagcacagccgccctgggctgcctggtgaaggactacttccccgagcccgtgaccgtgtcctggaacagcggcgctctgaccagcggcgtgcataccttccccgccgtgctccagagcagcggactgtactccctgagcagcgtggtgaccgtgccttccagcagcctgggcaccaagacctacacctgcaacgtggaccacaagcccagcaacaccaaggtggacaagagagtggagagcaagtacggccctccctgccccccttgccctgcccccgagttcgagggcggacctagcgtgttcctgttcccccccaagcccaaggacaccctgatgatcagcagaacccccgaggtgacctgcgtggtggtggacgtgtcccaggaggaccccgaggtccagtttaattggtacgtggacggcgtggaagtgcataacgccaagaccaagcccagagaggagcagttcaacagcacctacagagtggtgtccgtgctgaccgtgctgcaccaggactggctgaacggcaaggaatacaagtgcaaggtctccaacaagggcctggccagcagcatcgagaagaccatcagcaaggccaagggccagccacgggagccccaggtctgcaccctgccacctagccaagaggagatgaccaagaaccaggtgtccctgagctgtgccgtgaaaggcttctatcccagcgatatcgccgtggagtgggagagcaacggccagcccgagaacaactacaagaccaccccccctgtgctggacagcgacggcagcttcttcctggtttccaagctgaccgtggacaagtccagatggcaggagggcaacgtcttcagctgctccgtgatgcacgaggccctgcacaaccactacacccagaagtccctgagcctgagcctgggcaag

SEQ ID NO: 198 - protein, 214 aa, synthetic construct
DIQMTQSPSSLSASVGDRVTITCRASQNVGTNVAWYQKKPGKAPKALIYSASYRNSGVPSRFSGSGSGTDFTLTISSLQPEDFATYFCQQYNSYLLTFGGGTKVEIKRTVAAPSVFIFPPSDEQLKSGTASVVCLLNNFYPREAKVQWKVDNALQSGNSQESVTEQDSKDSTYSLSSTLTLSKADYEKHKVYACEVTHQGLSSPVTKSFNRGEC

SEQ ID NO: 199 - DNA, 642 bp, synthetic construct
  source 1..642: mol_type = other DNA
gacatccagatgacacagagccctagcagcctgtctgccagcgtgggagacagagtgaccatcacctgtagagccagccagaacgtgggcacaaacgtggcctggtatcagaagaagcctggcaaggcccctaaggctctgatctacagcgccagctacagaaacagcggcgtgccctctagattcagcggctctggctctggcaccgacttcaccctgacaatctctagcctgcagcctgaggacttcgctacctacttctgccagcagtacaacagctacctgctgaccttcggcggaggcaccaaggtggaaatcaagcgaactgtggctgcaccatctgtcttcatcttcccgccatctgatgagcagttgaaatctggaactgcctctgttgtgtgcctgctgaataacttctatcccagagaggccaaagtacagtggaaggtggataacgccctccaatcgggtaactcccaggagagtgtcacagagcaggacagcaaggacagcacctacagcctcagcagcaccctgacgctgagcaaagcagactacgagaaacacaaagtctacgcctgcgaagtcacccatcagggcctgagctcgcccgtcacaaagagcttcaacaggggagagtgt

SEQ ID NO: 200 - protein, 445 aa, synthetic construct
QVQLVQSGAEVKKPGSSVKVSCKASGYSFTGYTMNWVREAPGQGLEWMGLINPYNGGTRYNQKFQGRVTITADESTSTAYMELSSLRSEDTAVYYCARWALRYGMDYWGQGTLVTVSSASTKGPSVFPLAPCSRSTSESTAALGCLVKDYFPEPVTVSWNSGALTSGVHTFPAVLQSSGLYSLSSVVTVPSSSLGTKTYTCNVDHKPSNTKVDKRVESKYGPPCPPCPAPEFEGGPSVFLFPPKPKDTLMISRTPEVTCVVVDVSQEDPEVQFNWYVDGVEVHNAKTKPREEQFNSTYRVVSVLTVLHQDWLNGKEYKCKVSNKGLASSIEKTISKAKGQPREPQVCTLPPSQEEMTKNQVSLSCAVKGFYPSDIAVEWESNGQPENNYKTTPPVLDSDGSFFLVSKLTVDKSRWQEGNVFSCSVMHEALHNHYTQKSLSLSLGK

SEQ ID NO: 201 - DNA, 1335 bp, synthetic construct
  source 1..1335: mol_type = other DNA
caggttcagctggttcagtctggcgccgaagtgaagaaacctggcagcagcgtgaaggtgtcctgcaaggctagcggctacagcttcaccggctacaccatgaactgggtccgagaggctcctggacagggactcgaatggatgggcctgatcaacccttacaacggcggcaccagatacaaccagaaattccagggcagagtgaccattaccgcggacgagtctaccagcaccgcctacatggaactgagcagcctgagaagcgaggacaccgccgtgtactactgtgccagatgggctctgagatacggcatggactactggggccagggaaccctggttaccgttagctctgctagcaccaagggccccagcgtgttccccctggccccttgcagcagaagcaccagcgagagcacagccgccctgggctgcctggtgaaggactacttccccgagcccgtgaccgtgtcctggaacagcggcgctctgaccagcggcgtgcataccttccccgccgtgctccagagcagcggactgtactccctgagcagcgtggtgaccgtgccttccagcagcctgggcaccaagacctacacctgcaacgtggaccacaagcccagcaacaccaaggtggacaagagagtggagagcaagtacggccctccctgccccccttgccctgcccccgagttcgagggcggacctagcgtgttcctgttcccccccaagcccaaggacaccctgatgatcagcagaacccccgaggtgacctgcgtggtggtggacgtgtcccaggaggaccccgaggtccagtttaattggtacgtggacggcgtggaagtgcataacgccaagaccaagcccagagaggagcagttcaacagcacctacagagtggtgtccgtgctgaccgtgctgcaccaggactggctgaacggcaaggaatacaagtgcaaggtctccaacaagggcctggccagcagcatcgagaagaccatcagcaaggccaagggccagccacgggagccccaggtctgcaccctgccacctagccaagaggagatgaccaagaaccaggtgtccctgagctgtgccgtgaaaggcttctatcccagcgatatcgccgtggagtgggagagcaacggccagcccgagaacaactacaagaccaccccccctgtgctggacagcgacggcagcttcttcctggtttccaagctgaccgtggacaagtccagatggcaggagggcaacgtcttcagctgctccgtgatgcacgaggccctgcacaaccactacacccagaagtccctgagcctgagcctgggcaag

SEQ ID NO: 202 - protein, 118 aa, synthetic construct
QVQLVQSGAEVKKPGSSVKVSCKASGYSFTGYTMNWVREAPGQGLEWMGLINPYNGGTRYNQKFQGRVTITADESTSTAYMELSSLRSEDTAVYYCARWALRYGMDYWGQGTLVTVSS

SEQ ID NO: 203 - DNA, 354 bp, synthetic construct
  source 1..354: mol_type = other DNA
caggttcagctggttcagtctggcgccgaagtgaagaaacctggcagcagcgtgaaggtgtcctgcaaggctagcggctacagcttcaccggctacaccatgaactgggtccgagaggctcctggacagggactcgaatggatgggcctgatcaacccttacaacggcggcaccagatacaaccagaaattccagggcagagtgaccattaccgcggacgagtctaccagcaccgcctacatggaactgagcagcctgagaagcgaggacaccgccgtgtactactgtgccagatgggctctgagatacggcatggactactggggccagggaaccctggttaccgttagctct

SEQ ID NO: 204 - protein, 214 aa, synthetic construct
DIQMTQSPSSLSASVGDRVTITCQASQNVGTNVAWYQKKPGQAPKALIYSASYLNSGVPSRFSGSGSGTDFTFTISSLQPEDIATYFCQQYNSYLLTFGGGTKVEIKRTVAAPSVFIFPPSDEQLKSGTASVVCLLNNFYPREAKVQWKVDNALQSGNSQESVTEQDSKDSTYSLSSTLTLSKADYEKHKVYACEVTHQGLSSPVTKSFNRGEC

SEQ ID NO: 205 - DNA, 642 bp, synthetic construct
  source 1..642: mol_type = other DNA
gacatccagatgacacagagccctagcagcctgtctgccagcgtgggagacagagtgaccatcacctgtcaagccagccagaacgtgggcacaaacgtggcctggtatcagaagaagcctggccaggcccctaaggctctgatctacagcgccagctacttaaacagcggcgtgccctctagattcagcggctctggctctggcaccgacttcaccttcacaatctctagcctgcagcctgaggacatcgctacctacttctgccagcagtacaacagctacctgctgaccttcggcggaggcaccaaggtggaaatcaagcgaactgtggctgcaccatctgtcttcatcttcccgccatctgatgagcagttgaaatctggaactgcctctgttgtgtgcctgctgaataacttctatcccagagaggccaaagtacagtggaaggtggataacgccctccaatcgggtaactcccaggagagtgtcacagagcaggacagcaaggacagcacctacagcctcagcagcaccctgacgctgagcaaagcagactacgagaaacacaaagtctacgcctgcgaagtcacccatcagggcctgagctcgcccgtcacaaagagcttcaacaggggagagtgt

SEQ ID NO: 206 - protein, 107 aa, synthetic construct
DIQMTQSPSSLSASVGDRVTITCQASQNVGTNVAWYQKKPGQAPKALIYSASYLNSGVPSRFSGSGSGTDFTFTISSLQPEDIATYFCQQYNSYLLTFGGGTKVEIK

SEQ ID NO: 207 - DNA, 321 bp, synthetic construct
  source 1..321: mol_type = other DNA
gacatccagatgacacagagccctagcagcctgtctgccagcgtgggagacagagtgaccatcacctgtcaagccagccagaacgtgggcacaaacgtggcctggtatcagaagaagcctggccaggcccctaaggctctgatctacagcgccagctacttaaacagcggcgtgccctctagattcagcggctctggctctggcaccgacttcaccttcacaatctctagcctgcagcctgaggacatcgctacctacttctgccagcagtacaacagctacctgctgaccttcggcggaggcaccaaggtggaaatcaag

SEQ ID NO: 208 - protein, 11 aa, synthetic construct
QASQNVGTNVA

SEQ ID NO: 209 - protein, 7 aa, synthetic construct
SASYLNS

SEQ ID NO: 210 - protein, 214 aa, synthetic construct
DIQMTQSPSSLSASVGDRVTITCRASQNVGTNVAWYQKKPGQAPKALIYSASYLNSGVPSRFSGSGSGTDFTLTISSLQPEDFATYFCQQYNSYLLTFGGGTKVEIKRTVAAPSVFIFPPSDEQLKSGTASVVCLLNNFYPREAKVQWKVDNALQSGNSQESVTEQDSKDSTYSLSSTLTLSKADYEKHKVYACEVTHQGLSSPVTKSFNRGEC

SEQ ID NO: 211 - DNA, 642 bp, synthetic construct
  source 1..642: mol_type = other DNA
gacatccagatgacacagagccctagcagcctgtctgccagcgtgggagacagagtgaccatcacctgtagagccagccagaacgtgggcacaaacgtggcctggtatcagaagaagcctggccaggcccctaaggctctgatctacagcgccagctacttaaacagcggcgtgccctctagattcagcggctctggctctggcaccgacttcaccctgacaatctctagcctgcagcctgaggacttcgctacctacttctgccagcagtacaacagctacctgctgaccttcggcggaggcaccaaggtggaaatcaagcgaactgtggctgcaccatctgtcttcatcttcccgccatctgatgagcagttgaaatctggaactgcctctgttgtgtgcctgctgaataacttctatcccagagaggccaaagtacagtggaaggtggataacgccctccaatcgggtaactcccaggagagtgtcacagagcaggacagcaaggacagcacctacagcctcagcagcaccctgacgctgagcaaagcagactacgagaaacacaaagtctacgcctgcgaagtcacccatcagggcctgagctcgcccgtcacaaagagcttcaacaggggagagtgt

SEQ ID NO: 212 - protein, 107 aa, synthetic construct
DIQMTQSPSSLSASVGDRVTITCRASQNVGTNVAWYQKKPGQAPKALIYSASYLNSGVPSRFSGSGSGTDFTLTISSLQPEDFATYFCQQYNSYLLTFGGGTKVEIK

SEQ ID NO: 213 - DNA, 321 bp, synthetic construct
  source 1..321: mol_type = other DNA
gacatccagatgacacagagccctagcagcctgtctgccagcgtgggagacagagtgaccatcacctgtagagccagccagaacgtgggcacaaacgtggcctggtatcagaagaagcctggccaggcccctaaggctctgatctacagcgccagctacttaaacagcggcgtgccctctagattcagcggctctggctctggcaccgacttcaccctgacaatctctagcctgcagcctgaggacttcgctacctacttctgccagcagtacaacagctacctgctgaccttcggcggaggcaccaaggtggaaatcaag

SEQ ID NO: 214 - protein, 214 aa, synthetic construct
DIQMTQSPSSLSASVGDRVTITCQASQNVGTNVAWYQKKPGQAPKALIYSASYRNSGVPSRFSGSGSGTDFTFTISSLQPEDIATYFCQQYNSYLLTFGGGTKVEIKRTVAAPSVFIFPPSDEQLKSGTASVVCLLNNFYPREAKVQWKVDNALQSGNSQESVTEQDSKDSTYSLSSTLTLSKADYEKHKVYACEVTHQGLSSPVTKSFNRGEC

SEQ ID NO: 215 - DNA, 642 bp, synthetic construct
  source 1..642: mol_type = other DNA
gacatccagatgacacagagccctagcagcctgtctgccagcgtgggagacagagtgaccatcacctgtcaagccagccagaacgtgggcacaaacgtggcctggtatcagaagaagcctggccaggcccctaaggctctgatctacagcgccagctacagaaacagcggcgtgccctctagattcagcggctctggctctggcaccgacttcaccttcacaatctctagcctgcagcctgaggacatcgctacctacttctgccagcagtacaacagctacctgctgaccttcggcggaggcaccaaggtggaaatcaagcgaactgtggctgcaccatctgtcttcatcttcccgccatctgatgagcagttgaaatctggaactgcctctgttgtgtgcctgctgaataacttctatcccagagaggccaaagtacagtggaaggtggataacgccctccaatcgggtaactcccaggagagtgtcacagagcaggacagcaaggacagcacctacagcctcagcagcaccctgacgctgagcaaagcagactacgagaaacacaaagtctacgcctgcgaagtcacccatcagggcctgagctcgcccgtcacaaagagcttcaacaggggagagtgt

SEQ ID NO: 216 - protein, 107 aa, synthetic construct
DIQMTQSPSSLSASVGDRVTITCQASQNVGTNVAWYQKKPGQAPKALIYSASYRNSGVPSRFSGSGSGTDFTFTISSLQPEDIATYFCQQYNSYLLTFGGGTKVEIK

SEQ ID NO: 217 - DNA, 321 bp, synthetic construct
  source 1..321: mol_type = other DNA
gacatccagatgacacagagccctagcagcctgtctgccagcgtgggagacagagtgaccatcacctgtcaagccagccagaacgtgggcacaaacgtggcctggtatcagaagaagcctggccaggcccctaaggctctgatctacagcgccagctacagaaacagcggcgtgccctctagattcagcggctctggctctggcaccgacttcaccttcacaatctctagcctgcagcctgaggacatcgctacctacttctgccagcagtacaacagctacctgctgaccttcggcggaggcaccaaggtggaaatcaag

SEQ ID NO: 218 - protein, 214 aa, synthetic construct
DIQMTQSPSSLSASVGDRVTITCRASQNVGTNVAWYQKKPGQAPKALIYSASYRNSGVPSRFSGSGSGTDFTLTISSLQPEDFATYFCQQYNSYLLTFGGGTKVEIKRTVAAPSVFIFPPSDEQLKSGTASVVCLLNNFYPREAKVQWKVDNALQSGNSQESVTEQDSKDSTYSLSSTLTLSKADYEKHKVYACEVTHQGLSSPVTKSFNRGEC

SEQ ID NO: 219 - DNA, 642 bp, synthetic construct
  source 1..642: mol_type = other DNA
gacatccagatgacacagagccctagcagcctgtctgccagcgtgggagacagagtgaccatcacctgtagagccagccagaacgtgggcacaaacgtggcctggtatcagaagaagcctggccaggcccctaaggctctgatctacagcgccagctacagaaacagcggcgtgccctctagattcagcggctctggctctggcaccgacttcaccctgacaatctctagcctgcagcctgaggacttcgctacctacttctgccagcagtacaacagctacctgctgaccttcggcggaggcaccaaggtggaaatcaagcgaactgtggctgcaccatctgtcttcatcttcccgccatctgatgagcagttgaaatctggaactgcctctgttgtgtgcctgctgaataacttctatcccagagaggccaaagtacagtggaaggtggataacgccctccaatcgggtaactcccaggagagtgtcacagagcaggacagcaaggacagcacctacagcctcagcagcaccctgacgctgagcaaagcagactacgagaaacacaaagtctacgcctgcgaagtcacccatcagggcctgagctcgcccgtcacaaagagcttcaacaggggagagtgt

SEQ ID NO: 220 - protein, 107 aa, synthetic construct
DIQMTQSPSSLSASVGDRVTITCRASQNVGTNVAWYQKKPGQAPKALIYSASYRNSGVPSRFSGSGSGTDFTLTISSLQPEDFATYFCQQYNSYLLTFGGGTKVEIK

SEQ ID NO: 221 - DNA, 321 bp, synthetic construct
  source 1..321: mol_type = other DNA
gacatccagatgacacagagccctagcagcctgtctgccagcgtgggagacagagtgaccatcacctgtagagccagccagaacgtgggcacaaacgtggcctggtatcagaagaagcctggccaggcccctaaggctctgatctacagcgccagctacagaaacagcggcgtgccctctagattcagcggctctggctctggcaccgacttcaccctgacaatctctagcctgcagcctgaggacttcgctacctacttctgccagcagtacaacagctacctgctgaccttcggcggaggcaccaaggtggaaatcaag

SEQ ID NO: 222 - protein, 452 aa, synthetic construct
EVQLVESGGGLVQPGGSLRLSCAASGFTFNTYAMNWVRKAPGKGLEWVGRIRSKYNNYATYYADSVKDRFTISRDDSKNSLYLQMNSLKTEDTAVYYCVRHGNFGNSYVSWFAYWGQGTLVTVSSASTKGPSVFPLAPCSRSTSESTAALGCLVKDYFPEPVTVSWNSGALTSGVHTFPAVLQSSGLYSLSSVVTVPSSSLGTKTYTCNVDHKPSNTKVDKRVESKYGPPCPPCPAPEFEGGPSVFLFPPKPKDTLMISRTPEVTCVVVDVSQEDPEVQFNWYVDGVEVHNAKTKPREEQFNSTYRVVSVLTVLHQDWLNGKEYKCKVSNKGLASSIEKTISKAKGQPREPQVYTLPPCQEEMTKNQVSLWCLVKGFYPSDIAVEWESNGQPENNYKTTPPVLDSDGSFFLYSKLTVDKSRWQEGNVFSCSVMHEALHNHYTQKSLSLSLGK

SEQ ID NO: 223 - DNA, 1356 bp, synthetic construct
  source 1..1356: mol_type = other DNA
gaggtgcagctggttgaatctggcggaggactggttcagcctggcggatctctgagactgtcttgtgccgccagcggcttcaccttcaacacctacgctatgaactgggtccgaaaggcccctggcaaaggactggaatgggtgggaagaatcaggtccaagtacaacaactacgccacctactacgccgacagcgtgaaggacagattcaccatcagcagggacgacagcaagaacagcctgtacctgcagatgaacagcctgaaaaccgaggacaccgccgtgtactactgtgtcagacacggcaacttcggcaacagctatgtgtcttggtttgcctactggggccagggcacactggtcacagttagctctgctagcaccaagggccccagcgtgttccccctggccccttgcagcagaagcaccagcgagagcacagccgccctgggctgcctggtgaaggactacttccccgagcccgtgaccgtgtcctggaacagcggcgctctgaccagcggcgtgcataccttccccgccgtgctccagagcagcggactgtactccctgagcagcgtggtgaccgtgccttccagcagcctgggcaccaagacctacacctgcaacgtggaccacaagcccagcaacaccaaggtggacaagagagtggagagcaagtacggccctccctgccccccttgccctgcccccgagttcgagggcggacctagcgtgttcctgttcccccccaagcccaaggacaccctgatgatcagcagaacccccgaggtgacctgcgtggtggtggacgtgtcccaggaggaccccgaggtccagtttaattggtacgtggacggcgtggaagtgcataacgccaagaccaagcccagagaggagcagttcaacagcacctacagagtggtgtccgtgctgaccgtgctgcaccaggactggctgaacggcaaggaatacaagtgcaaggtctccaacaagggcctggccagcagcatcgagaagaccatcagcaaggccaagggccagccacgggagccccaggtctacaccctgccaccttgtcaagaggagatgaccaagaaccaggtgtccctgtggtgtctggtgaaaggcttctatcccagcgatatcgccgtggagtgggagagcaacggccagcccgagaacaactacaagaccaccccccctgtgctggacagcgacggcagcttcttcctgtactccaagctgaccgtggacaagtccagatggcaggagggcaacgtcttcagctgctccgtgatgcacgaggccctgcacaaccactacacccagaagtccctgagcctgagcctgggcaag

SEQ ID NO: 224 - protein, 215 aa, synthetic construct
QAVVTQEPSLTVSPGGTVTLTCRSSTGAVTTSNYANWVQEKPGQAPRGLIGGTNKRAPWTPARFSGSLLGGKAALTITGAQAEDEAEYYCVLWYSNLWVFGGGTKLTVLGQPKAAPSVTLFPPSSEELQANKATLVCLISDFYPGAVTVAWKADSSPVKAGVETTTPSKQSNNKYAASSYLSLTPEQWKSHRSYSCQVTHEGSTVEKTVAPTECS

SEQ ID NO: 225 - DNA, 645 bp, synthetic construct
  source 1..645: mol_type = other DNA
caggctgtggtcacacaagagcctagcctgacagtgtctcctggcggcacagtgaccctgacctgtagatcttctacaggcgccgtgaccaccagcaactacgctaattgggtgcaggagaagcccggccaggctcctagaggactgatcggcggaacaaacaagagagccccttggacacccgccagattctctggatctctgctcggcggaaaggccgctctgacaatcactggtgctcaggctgaggacgaggccgagtactattgtgtgctgtggtacagcaacctgtgggtgttcggcggaggcaccaaactgacagttctgggtcagcccaaggcggcgccctcggtcactctgttcccgccctcctctgaggagcttcaagccaacaaggccacactggtgtgtctcataagtgacttctatccgggagccgtgacagtggcctggaaggcagatagcagccccgtcaaggcgggagtggagaccaccacaccctccaaacaaagcaacaacaagtacgcggccagcagctacctgagcctgacgcctgagcagtggaagtcccacagaagctacagctgccaggtcacgcatgaagggagcaccgtggagaagacagtggcccctacagaatgttca

SEQ ID NO: 226 - protein, 218 aa, synthetic construct
DIVLTQSPASLAVSPGQRATITCRASKSVSTSGYSYMHWYQKKPGQPPKLLIYLASNLESGVPARFSGSGSGTDFTLTINPVEAEDTANYYCQHSRELPWTFGQGTKVEIKRTVAAPSVFIFPPSDEQLKSGTASVVCLLNNFYPREAKVQWKVDNALQSGNSQESVTEQDSKDSTYSLSSTLTLSKADYEKHKVYACEVTHQGLSSPVTKSFNRGEC

SEQ ID NO: 227 - DNA, 654 bp, synthetic construct
  source 1..654: mol_type = other DNA
gacatcgtgctgacacagagccctgcttctctggctgtgtctcctggccagagagccaccatcacctgtagagccagcaagagcgtgtccaccagcggctactcttacatgcactggtatcagaagaagcccggccagcctcctaagctgctgatctacctggctagcaacctcgaaagcggagtgcctgctagattttctggcagcggctctggcaccgacttcaccctgacaatcaaccccgtggaagccgaagacaccgccaactactactgccagcacagcagagagctgccctggacatttggccagggcaccaaggtggaaatcaagcgaactgtggctgcaccatctgtcttcatcttcccgccatctgatgagcagttgaaatctggaactgcctctgttgtgtgcctgctgaataacttctatcccagagaggccaaagtacagtggaaggtggataacgccctccaatcgggtaactcccaggagagtgtcacagagcaggacagcaaggacagcacctacagcctcagcagcaccctgacgctgagcaaagcagactacgagaaacacaaagtctacgcctgcgaagtcacccatcagggcctgagctcgcccgtcacaaagagcttcaacaggggagagtgt

SEQ ID NO: 228 - protein, 704 aa, synthetic construct
DIQMTQSPSSLSASVGDRVTITCQASQNVGTNVAWYQQKPGQAPKALIYSASYLNSGVPSRFSGSGSGTDFTFTISSLQPEDIATYFCQQYNSYLLTFGCGTKVEIKGGGGSGGGGSGGGGSQVQLVQSGAEVKKPGSSVKVSCKASGYSFTGYTMNWVRQAPGQCLEWMGLINPYNGGTRYNQKFQGRVTITADESTSTAYMELSSLRSEDTAVYYCARWALRYGMDYWGQGTLVTVSSGGGGSGGGGSGGGGSQVQLVQSGSELKKPGASVKVSCKASGYIFTNFGMNWVREAPGQGLEWMGWINTYTGEQIYADGFTGRFVFSLDTSVSTAYLQISSLKAEDTAVYFCARGEIYYGYDVGFVYWGQGTLVTVSSASTKGPSVFPLAPCSRSTSESTAALGCLVKDYFPEPVTVSWNSGALTSGVHTFPAVLQSSGLYSLSSVVTVPSSSLGTKTYTCNVDHKPSNTKVDKRVESKYGPPCPPCPAPEFEGGPSVFLFPPKPKDTLMISRTPEVTCVVVDVSQEDPEVQFNWYVDGVEVHNAKTKPREEQFNSTYRVVSVLTVLHQDWLNGKEYKCKVSNKGLASSIEKTISKAKGQPREPQVCTLPPSQEEMTKNQVSLSCAVKGFYPSDIAVEWESNGQPENNYKTTPPVLDSDGSFFLVSKLTVDKSRWQEGNVFSCSVMHEALHNHYTQKSLSLSLGK

SEQ ID NO: 229 - DNA, 2112 bp, synthetic construct
  source 1..2112: mol_type = other DNA
gacatccagatgacacagagccctagcagcctgtctgccagcgtgggagacagagtgaccatcacctgtcaagccagccagaacgtgggcacaaacgtggcctggtatcagcagaagcctggccaggcccctaaggctctgatctacagcgccagctacttaaacagcggcgtgccctctagattcagcggctctggctctggcaccgacttcaccttcacaatctctagcctgcagcctgaggacatcgctacctacttctgccagcagtacaacagctacctgctgaccttcggctgcggcaccaaggtggaaatcaagggaggcggaggatctggtggcggaggaagcggtggcggcggatcccaggttcagctggttcagtctggcgccgaagtgaagaaacctggcagcagcgtgaaggtgtcctgcaaggctagcggctacagcttcaccggctacaccatgaactgggtccgacaggctcctggacagtgcctcgaatggatgggcctgatcaacccttacaacggcggcaccagatacaaccagaaattccagggcagagtgaccattaccgcggacgagtctaccagcaccgcctacatggaactgagcagcctgagaagcgaggacaccgccgtgtactactgtgccagatgggctctgagatacggcatggactactggggccagggaaccctggttaccgttagctctggaggcggaggatctggtggcggaggaagcggtggcggcggatcccaggttcagctggtgcagtctggcagcgagctgaagaaacctggcgcctctgtgaaggtgtcctgcaaggctagcggctacatcttcaccaacttcggcatgaactgggtccgagaggctcctggacagggactcgaatggatgggctggatcaacacctacaccggcgagcagatctacgccgatggcttcacaggcagattcgtgttcagcctggacaccagcgtcagcacagcttacctgcagatcagctctctgaaggccgaggataccgccgtgtacttctgtgccagaggcgagatctactacggctacgacgtgggctttgtgtactggggccagggaacactggtcaccgttagctctgctagcaccaagggccccagcgtgttccccctggccccttgcagcagaagcaccagcgagagcacagccgccctgggctgcctggtgaaggactacttccccgagcccgtgaccgtgtcctggaacagcggcgctctgaccagcggcgtgcataccttccccgccgtgctccagagcagcggactgtactccctgagcagcgtggtgaccgtgccttccagcagcctgggcaccaagacctacacctgcaacgtggaccacaagcccagcaacaccaaggtggacaagagagtggagagcaagtacggccctccctgccccccttgccctgcccccgagttcgagggcggacctagcgtgttcctgttcccccccaagcccaaggacaccctgatgatcagcagaacccccgaggtgacctgcgtggtggtggacgtgtcccaggaggaccccgaggtccagtttaattggtacgtggacggcgtggaagtgcataacgccaagaccaagcccagagaggagcagttcaacagcacctacagagtggtgtccgtgctgaccgtgctgcaccaggactggctgaacggcaaggaatacaagtgcaaggtctccaacaagggcctggccagcagcatcgagaagaccatcagcaaggccaagggccagccacgggagccccaggtctgcaccctgccacctagccaagaggagatgaccaagaaccaggtgtccctgagctgtgccgtgaaaggcttctatcccagcgatatcgccgtggagtgggagagcaacggccagcccgagaacaactacaagaccaccccccctgtgctggacagcgacggcagcttcttcctggtttccaagctgaccgtggacaagtccagatggcaggagggcaacgtcttcagctgctccgtgatgcacgaggccctgcacaaccactacacccagaagtccctgagcctgagcctgggcaag

SEQ ID NO: 230 - protein, 107 aa, synthetic construct
DIQMTQSPSSLSASVGDRVTITCQASQNVGTNVAWYQQKPGQAPKALIYSASYLNSGVPSRFSGSGSGTDFTFTISSLQPEDIATYFCQQYNSYLLTFGCGTKVEIK

SEQ ID NO: 231 - protein, 15 aa, synthetic construct
GGGGSGGGGSGGGGS

SEQ ID NO: 232 - protein, 118 aa, synthetic construct
QVQLVQSGAEVKKPGSSVKVSCKASGYSFTGYTMNWVRQAPGQCLEWMGLINPYNGGTRYNQKFQGRVTITADESTSTAYMELSSLRSEDTAVYYCARWALRYGMDYWGQGTLVTVSS

SEQ ID NO: 233 - protein, 122 aa, synthetic construct
QVQLVQSGSELKKPGASVKVSCKASGYIFTNFGMNWVREAPGQGLEWMGWINTYTGEQIYADGFTGRFVFSLDTSVSTAYLQISSLKAEDTAVYFCARGEIYYGYDVGFVYWGQGTLVTVSS

SEQ ID NO: 234 - protein, 704 aa, synthetic construct
QVQLVQSGAEVKKPGSSVKVSCKASGYSFTGYTMNWVRQAPGQCLEWMGLINPYNGGTRYNQKFQGRVTITADESTSTAYMELSSLRSEDTAVYYCARWALRYGMDYWGQGTLVTVSSGGGGSGGGGSGGGGSDIQMTQSPSSLSASVGDRVTITCQASQNVGTNVAWYQQKPGQAPKALIYSASYLNSGVPSRFSGSGSGTDFTFTISSLQPEDIATYFCQQYNSYLLTFGCGTKVEIKGGGGSGGGGSGGGGSQVQLVQSGSELKKPGASVKVSCKASGYIFTNFGMNWVREAPGQGLEWMGWINTYTGEQIYADGFTGRFVFSLDTSVSTAYLQISSLKAEDTAVYFCARGEIYYGYDVGFVYWGQGTLVTVSSASTKGPSVFPLAPCSRSTSESTAALGCLVKDYFPEPVTVSWNSGALTSGVHTFPAVLQSSGLYSLSSVVTVPSSSLGTKTYTCNVDHKPSNTKVDKRVESKYGPPCPPCPAPEFEGGPSVFLFPPKPKDTLMISRTPEVTCVVVDVSQEDPEVQFNWYVDGVEVHNAKTKPREEQFNSTYRVVSVLTVLHQDWLNGKEYKCKVSNKGLASSIEKTISKAKGQPREPQVCTLPPSQEEMTKNQVSLSCAVKGFYPSDIAVEWESNGQPENNYKTTPPVLDSDGSFFLVSKLTVDKSRWQEGNVFSCSVMHEALHNHYTQKSLSLSLGK

SEQ ID NO: 235 - DNA, 2112 bp, synthetic construct
  source 1..2112: mol_type = other DNA
caggttcagctggttcagtctggcgccgaagtgaagaaacctggcagcagcgtgaaggtgtcctgcaaggctagcggctacagcttcaccggctacaccatgaactgggtccgacaggctcctggacagtgcctcgaatggatgggcctgatcaacccttacaacggcggcaccagatacaaccagaaattccagggcagagtgaccattaccgcggacgagtctaccagcaccgcctacatggaactgagcagcctgagaagcgaggacaccgccgtgtactactgtgccagatgggctctgagatacggcatggactactggggccagggaaccctggttaccgttagctctggaggcggaggatctggtggcggaggaagcggtggcggcggatccgacatccagatgacacagagccctagcagcctgtctgccagcgtgggagacagagtgaccatcacctgtcaagccagccagaacgtgggcacaaacgtggcctggtatcagcagaagcctggccaggcccctaaggctctgatctacagcgccagctacttaaacagcggcgtgccctctagattcagcggctctggctctggcaccgacttcaccttcacaatctctagcctgcagcctgaggacatcgctacctacttctgccagcagtacaacagctacctgctgaccttcggctgcggcaccaaggtggaaatcaagggaggcggaggatctggtggcggaggaagcggtggcggcggatcccaggttcagctggtgcagtctggcagcgagctgaagaaacctggcgcctctgtgaaggtgtcctgcaaggctagcggctacatcttcaccaacttcggcatgaactgggtccgagaggctcctggacagggactcgaatggatgggctggatcaacacctacaccggcgagcagatctacgccgatggcttcacaggcagattcgtgttcagcctggacaccagcgtcagcacagcttacctgcagatcagctctctgaaggccgaggataccgccgtgtacttctgtgccagaggcgagatctactacggctacgacgtgggctttgtgtactggggccagggaacactggtcaccgttagctctgctagcaccaagggccccagcgtgttccccctggccccttgcagcagaagcaccagcgagagcacagccgccctgggctgcctggtgaaggactacttccccgagcccgtgaccgtgtcctggaacagcggcgctctgaccagcggcgtgcataccttccccgccgtgctccagagcagcggactgtactccctgagcagcgtggtgaccgtgccttccagcagcctgggcaccaagacctacacctgcaacgtggaccacaagcccagcaacaccaaggtggacaagagagtggagagcaagtacggccctccctgccccccttgccctgcccccgagttcgagggcggacctagcgtgttcctgttcccccccaagcccaaggacaccctgatgatcagcagaacccccgaggtgacctgcgtggtggtggacgtgtcccaggaggaccccgaggtccagtttaattggtacgtggacggcgtggaagtgcataacgccaagaccaagcccagagaggagcagttcaacagcacctacagagtggtgtccgtgctgaccgtgctgcaccaggactggctgaacggcaaggaatacaagtgcaaggtctccaacaagggcctggccagcagcatcgagaagaccatcagcaaggccaagggccagccacgggagccccaggtctgcaccctgccacctagccaagaggagatgaccaagaaccaggtgtccctgagctgtgccgtgaaaggcttctatcccagcgatatcgccgtggagtgggagagcaacggccagcccgagaacaactacaagaccaccccccctgtgctggacagcgacggcagcttcttcctggtttccaagctgaccgtggacaagtccagatggcaggagggcaacgtcttcagctgctccgtgatgcacgaggccctgcacaaccactacacccagaagtccctgagcctgagcctgggcaag

SEQ ID NO: 236 - protein, 707 aa, synthetic construct
DIQMTQSPSSLSASVGDRVTITCQASQNVGTNVAWYQQKPGQAPKALIYSASYLNSGVPSRFSGSGSGTDFTFTISSLQPEDIATYFCQQYNSYLLTFGCGTKVEIKGGGGSGGGGSGGGGSQVQLVQSGAEVKKPGSSVKVSCKASGYSFTGYTMNWVRQAPGQCLEWMGLINPYNGGTRYNQKFQGRVTITADESTSTAYMELSSLRSEDTAVYYCARWALRYGMDYWGQGTLVTVSSGGGGSGGGGSGGGGSEVQLVESGGGLVQPGGSLRLSCAASGFTFNTYAMNWVRKAPGKGLEWVGRIRSKYNNYATYYADSVKDRFTISRDDSKNSLYLQMNSLKTEDTAVYYCVRHGNFGNSYVSWFAYWGQGTLVTVSSASTKGPSVFPLAPCSRSTSESTAALGCLVKDYFPEPVTVSWNSGALTSGVHTFPAVLQSSGLYSLSSVVTVPSSSLGTKTYTCNVDHKPSNTKVDKRVESKYGPPCPPCPAPEFEGGPSVFLFPPKPKDTLMISRTPEVTCVVVDVSQEDPEVQFNWYVDGVEVHNAKTKPREEQFNSTYRVVSVLTVLHQDWLNGKEYKCKVSNKGLASSIEKTISKAKGQPREPQVYTLPPCQEEMTKNQVSLWCLVKGFYPSDIAVEWESNGQPENNYKTTPPVLDSDGSFFLYSKLTVDKSRWQEGNVFSCSVMHEALHNHYTQKSLSLSLGK

SEQ ID NO: 237 - DNA, 2121 bp, synthetic construct
  source 1..2121: mol_type = other DNA
gacatccagatgacacagagccctagcagcctgtctgccagcgtgggagacagagtgaccatcacctgtcaagccagccagaacgtgggcacaaacgtggcctggtatcagcagaagcctggccaggcccctaaggctctgatctacagcgccagctacttaaacagcggcgtgccctctagattcagcggctctggctctggcaccgacttcaccttcacaatctctagcctgcagcctgaggacatcgctacctacttctgccagcagtacaacagctacctgctgaccttcggctgcggcaccaaggtggaaatcaagggaggcggaggatctggtggcggaggaagcggtggcggcggatcccaggttcagctggttcagtctggcgccgaagtgaagaaacctggcagcagcgtgaaggtgtcctgcaaggctagcggctacagcttcaccggctacaccatgaactgggtccgacaggctcctggacagtgcctcgaatggatgggcctgatcaacccttacaacggcggcaccagatacaaccagaaattccagggcagagtgaccattaccgcggacgagtctaccagcaccgcctacatggaactgagcagcctgagaagcgaggacaccgccgtgtactactgtgccagatgggctctgagatacggcatggactactggggccagggaaccctggttaccgttagctctggaggcggaggatctggtggcggaggaagcggtggcggcggatccgaggtgcagctggttgaatctggcggaggactggttcagcctggcggatctctgagactgtcttgtgccgccagcggcttcaccttcaacacctacgctatgaactgggtccgaaaggcccctggcaaaggactggaatgggtgggaagaatcaggtccaagtacaacaactacgccacctactacgccgacagcgtgaaggacagattcaccatcagcagggacgacagcaagaacagcctgtacctgcagatgaacagcctgaaaaccgaggacaccgccgtgtactactgtgtcagacacggcaacttcggcaacagctatgtgtcttggtttgcctactggggccagggcacactggtcacagttagctctgctagcaccaagggccccagcgtgttccccctggccccttgcagcagaagcaccagcgagagcacagccgccctgggctgcctggtgaaggactacttccccgagcccgtgaccgtgtcctggaacagcggcgctctgaccagcggcgtgcataccttccccgccgtgctccagagcagcggactgtactccctgagcagcgtggtgaccgtgccttccagcagcctgggcaccaagacctacacctgcaacgtggaccacaagcccagcaacaccaaggtggacaagagagtggagagcaagtacggccctccctgccccccttgccctgcccccgagttcgagggcggacctagcgtgttcctgttcccccccaagcccaaggacaccctgatgatcagcagaacccccgaggtgacctgcgtggtggtggacgtgtcccaggaggaccccgaggtccagtttaattggtacgtggacggcgtggaagtgcataacgccaagaccaagcccagagaggagcagttcaacagcacctacagagtggtgtccgtgctgaccgtgctgcaccaggactggctgaacggcaaggaatacaagtgcaaggtctccaacaagggcctggccagcagcatcgagaagaccatcagcaaggccaagggccagccacgggagccccaggtctacaccctgccaccttgtcaagaggagatgaccaagaaccaggtgtccctgtggtgtctggtgaaaggcttctatcccagcgatatcgccgtggagtgggagagcaacggccagcccgagaacaactacaagaccaccccccctgtgctggacagcgacggcagcttcttcctgtactccaagctgaccgtggacaagtccagatggcaggagggcaacgtcttcagctgctccgtgatgcacgaggccctgcacaaccactacacccagaagtccctgagcctgagcctgggcaag

SEQ ID NO: 238 - DNA, 1347 bp, synthetic construct
  source 1..1347: mol_type = other DNA
caggttcagctggtgcagtctggcagcgagctgaagaaacctggcgcctctgtgaaggtgtcctgcaaggctagcggctacatcttcaccaacttcggcatgaactgggtccgagaggctcctggacagggactcgaatggatgggctggatcaacacctacaccggcgagcagatctacgccgatggcttcacaggcagattcgtgttcagcctggacaccagcgtcagcacagcttacctgcagatcagctctctgaaggccgaggataccgccgtgtacttctgtgccagaggcgagatctactacggctacgacgtgggctttgtgtactggggccagggaacactggtcaccgttagctctgctagcaccaagggccccagcgtgttccccctggccccttgcagcagaagcaccagcgagagcacagccgccctgggctgcctggtgaaggactacttccccgagcccgtgaccgtgtcctggaacagcggcgctctgaccagcggcgtgcataccttccccgccgtgctccagagcagcggactgtactccctgagcagcgtggtgaccgtgccttccagcagcctgggcaccaagacctacacctgcaacgtggaccacaagcccagcaacaccaaggtggacaagagagtggagagcaagtacggccctccctgccccccttgccctgcccccgagttcgagggcggacctagcgtgttcctgttcccccccaagcccaaggacaccctgatgatcagcagaacccccgaggtgacctgcgtggtggtggacgtgtcccaggaggaccccgaggtccagtttaattggtacgtggacggcgtggaagtgcataacgccaagaccaagcccagagaggagcagttcaacagcacctacagagtggtgtccgtgctgaccgtgctgcaccaggactggctgaacggcaaggaatacaagtgcaaggtctccaacaagggcctggccagcagcatcgagaagaccatcagcaaggccaagggccagccacgggagccccaggtctgcaccctgccacctagccaagaggagatgaccaagaaccaggtgtccctgagctgtgccgtgaaaggcttctatcccagcgatatcgccgtggagtgggagagcaacggccagcccgagaacaactacaagaccaccccccctgtgctggacagcgacggcagcttcttcctggtttccaagctgaccgtggacaagtccagatggcaggagggcaacgtcttcagctgctccgtgatgcacgaggccctgcacaaccactacacccagaagtccctgagcctgagcctgggcaag

SEQ ID NO: 239 - protein, 707 aa, synthetic construct
QVQLVQSGAEVKKPGSSVKVSCKASGYSFTGYTMNWVRQAPGQCLEWMGLINPYNGGTRYNQKFQGRVTITADESTSTAYMELSSLRSEDTAVYYCARWALRYGMDYWGQGTLVTVSSGGGGSGGGGSGGGGSDIQMTQSPSSLSASVGDRVTITCQASQNVGTNVAWYQQKPGQAPKALIYSASYLNSGVPSRFSGSGSGTDFTFTISSLQPEDIATYFCQQYNSYLLTFGCGTKVEIKGGGGSGGGGSGGGGSEVQLVESGGGLVQPGGSLRLSCAASGFTFNTYAMNWVRKAPGKGLEWVGRIRSKYNNYATYYADSVKDRFTISRDDSKNSLYLQMNSLKTEDTAVYYCVRHGNFGNSYVSWFAYWGQGTLVTVSSASTKGPSVFPLAPCSRSTSESTAALGCLVKDYFPEPVTVSWNSGALTSGVHTFPAVLQSSGLYSLSSVVTVPSSSLGTKTYTCNVDHKPSNTKVDKRVESKYGPPCPPCPAPEFEGGPSVFLFPPKPKDTLMISRTPEVTCVVVDVSQEDPEVQFNWYVDGVEVHNAKTKPREEQFNSTYRVVSVLTVLHQDWLNGKEYKCKVSNKGLASSIEKTISKAKGQPREPQVYTLPPCQEEMTKNQVSLWCLVKGFYPSDIAVEWESNGQPENNYKTTPPVLDSDGSFFLYSKLTVDKSRWQEGNVFSCSVMHEALHNHYTQKSLSLSLGK

SEQ ID NO: 240 - DNA, 2121 bp, synthetic construct
  source 1..2121: mol_type = other DNA
caggttcagctggttcagtctggcgccgaagtgaagaaacctggcagcagcgtgaaggtgtcctgcaaggctagcggctacagcttcaccggctacaccatgaactgggtccgacaggctcctggacagtgcctcgaatggatgggcctgatcaacccttacaacggcggcaccagatacaaccagaaattccagggcagagtgaccattaccgcggacgagtctaccagcaccgcctacatggaactgagcagcctgagaagcgaggacaccgccgtgtactactgtgccagatgggctctgagatacggcatggactactggggccagggaaccctggttaccgttagctctggaggcggaggatctggtggcggaggaagcggtggcggcggatccgacatccagatgacacagagccctagcagcctgtctgccagcgtgggagacagagtgaccatcacctgtcaagccagccagaacgtgggcacaaacgtggcctggtatcagcagaagcctggccaggcccctaaggctctgatctacagcgccagctacttaaacagcggcgtgccctctagattcagcggctctggctctggcaccgacttcaccttcacaatctctagcctgcagcctgaggacatcgctacctacttctgccagcagtacaacagctacctgctgaccttcggctgcggcaccaaggtggaaatcaagggaggcggaggatctggtggcggaggaagcggtggcggcggatccgaggtgcagctggttgaatctggcggaggactggttcagcctggcggatctctgagactgtcttgtgccgccagcggcttcaccttcaacacctacgctatgaactgggtccgaaaggcccctggcaaaggactggaatgggtgggaagaatcaggtccaagtacaacaactacgccacctactacgccgacagcgtgaaggacagattcaccatcagcagggacgacagcaagaacagcctgtacctgcagatgaacagcctgaaaaccgaggacaccgccgtgtactactgtgtcagacacggcaacttcggcaacagctatgtgtcttggtttgcctactggggccagggcacactggtcacagttagctctgctagcaccaagggccccagcgtgttccccctggccccttgcagcagaagcaccagcgagagcacagccgccctgggctgcctggtgaaggactacttccccgagcccgtgaccgtgtcctggaacagcggcgctctgaccagcggcgtgcataccttccccgccgtgctccagagcagcggactgtactccctgagcagcgtggtgaccgtgccttccagcagcctgggcaccaagacctacacctgcaacgtggaccacaagcccagcaacaccaaggtggacaagagagtggagagcaagtacggccctccctgccccccttgccctgcccccgagttcgagggcggacctagcgtgttcctgttcccccccaagcccaaggacaccctgatgatcagcagaacccccgaggtgacctgcgtggtggtggacgtgtcccaggaggaccccgaggtccagtttaattggtacgtggacggcgtggaagtgcataacgccaagaccaagcccagagaggagcagttcaacagcacctacagagtggtgtccgtgctgaccgtgctgcaccaggactggctgaacggcaaggaatacaagtgcaaggtctccaacaagggcctggccagcagcatcgagaagaccatcagcaaggccaagggccagccacgggagccccaggtctacaccctgccaccttgtcaagaggagatgaccaagaaccaggtgtccctgtggtgtctggtgaaaggcttctatcccagcgatatcgccgtggagtgggagagcaacggccagcccgagaacaactacaagaccaccccccctgtgctggacagcgacggcagcttcttcctgtactccaagctgaccgtggacaagtccagatggcaggagggcaacgtcttcagctgctccgtgatgcacgaggccctgcacaaccactacacccagaagtccctgagcctgagcctgggcaag

SEQ ID NO: 241 - protein, 6 aa, synthetic construct
TSYTMY

SEQ ID NO: 242 - protein, 17 aa, synthetic construct
  MOD_RES 14: note = Xaa=K or N
  MOD_RES 16: note = Xaa=K or Q
  MOD_RES 17: note = Xaa=A or G
YIYPGNGGTNYNQXFXX

SEQ ID NO: 243 - protein, 10 aa, synthetic construct
  MOD_RES 1: note = Xaa=S or R
  MOD_RES 7: note = Xaa=S or R
  MOD_RES 8: note = Xaa=Y or F
XASSSVXXMH

SEQ ID NO: 244 - protein, 7 aa, synthetic construct
  MOD_RES 6: note = Xaa=V or L
DTSKXAS

SEQ ID NO: 245 - protein, 9 aa, synthetic construct
  MOD_RES 4: note = Xaa=S or N
  MOD_RES 5: note = Xaa=S or N
  MOD_RES 6: note = Xaa=N or Y or K
  MOD_RES 8: note = Xaa=L or P
QQWXXXPXT

SEQ ID NO: 246 - protein, 17 aa, synthetic construct
  MOD_RES 9: note = Xaa=S or T
  MOD_RES 10: note = Xaa=R or S or N
  MOD_RES 13: note = Xaa=Q or L
  MOD_RES 16: note = Xaa=K or Q
LINPYNGGXXYNXKFXG

SEQ ID NO: 247 - protein, 9 aa, synthetic construct
  MOD_RES 1: note = Xaa=W or L
  MOD_RES 2: note = Xaa=A or P or G
  MOD_RES 3: note = Xaa=I or L
  MOD_RES 5: note = Xaa=Y or N
  MOD_RES 6: note = Xaa=A or G
XXXRXXMDY

SEQ ID NO: 248 - protein, 11 aa, synthetic construct
  MOD_RES 1: note = Xaa=K or R or Q
  MOD_RES 5: note = Xaa=N or S
  MOD_RES 6: note = Xaa=V or I
  MOD_RES 7: note = Xaa=G or S
  MOD_RES 8: note = Xaa=T or N
  MOD_RES 10: note = Xaa=V or L
  MOD_RES 11: note = Xaa=A or H
XASQXXXXNXX

SEQ ID NO: 249 - skipped

SEQ ID NO: 250 - protein, 9 aa, synthetic construct
  MOD_RES 3: note = Xaa=Y or S
  MOD_RES 6: note = Xaa=Y or W
  MOD_RES 7: note = Xaa=L or P
  MOD_RES 8: note = Xaa=L or Q
QQXNSXXXT

SEQ ID NO: 251 - protein, 17 aa, synthetic construct
  MOD_RES 16: note = Xaa=K or Q
NFHPYNDVTKYNEKFXG

SEQ ID NO: 252 - protein, 6 aa, synthetic construct
  MOD_RES 4: note = Xaa=Y or T
TSYXMY

SEQ ID NO: 253 - protein, 17 aa, synthetic construct
  MOD_RES 1: note = Xaa=G or Y
  MOD_RES 6: note = Xaa=N or S
  MOD_RES 8: note = Xaa=G or Y
  MOD_RES 10: note = Xaa=K or N
  MOD_RES 13: note = Xaa=Q or E
  MOD_RES 16: note = Xaa=K or Q
  MOD_RES 17: note = Xaa=S or D or G
XINPSXGXTXYNXKFXX

SEQ ID NO: 254 - protein, 14 aa, synthetic construct
  MOD_RES 1: note = Xaa=G or W
  MOD_RES 2: note = Xaa=G or S
  MOD_RES 3: note = Xaa=G or L
  MOD_RES 4: note = Xaa=R or N
  MOD_RES 5: note = Xaa=E or S
  MOD_RES 6: note = Xaa=Y or R
  MOD_RES 7: note = Xaa=Y or L
  MOD_RES 9: note = Xaa=A or Y
  MOD_RES 10: note = Xaa=Y or M
  MOD_RES 11: note = Xaa=A or inexistence
  MOD_RES 12: note = Xaa=M or inexistence
XXXXXXXYXXXXDY

SEQ ID NO: 255 - protein, 11 aa, synthetic construct
  MOD_RES 1: note = Xaa=R or Q or S
  MOD_RES 4: note = Xaa=Q or S
  MOD_RES 5: note = Xaa=D or S
  MOD_RES 6: note = Xaa=I or V
  MOD_RES 7: note = Xaa=S or inexistence
  MOD_RES 8: note = Xaa=N or S
  MOD_RES 10: note = Xaa=L or M
  MOD_RES 11: note = Xaa=N or Y
XASXXXXXYXX

SEQ ID NO: 256 - protein, 7 aa, synthetic construct
  MOD_RES 1: note = Xaa=Y or G
  MOD_RES 4: note = Xaa= R or N
  MOD_RES 6: note = Xaa=H or A
XTSXLXS

SEQ ID NO: 257 - protein, 9 aa, synthetic construct
  MOD_RES 3: note = Xaa=R or G
  MOD_RES 4: note = Xaa=Y or S
  MOD_RES 6: note = Xaa=L or Y
  MOD_RES 8: note = Xaa=Y or L
QQXXSXPXT

SEQ ID NO: 258 - protein, 6 aa, synthetic construct
  MOD_RES 2: note = Xaa=S or N
  MOD_RES 6: note = Xaa=Y or H
TXYVMX

SEQ ID NO: 259 - protein, 17 aa, synthetic construct
  MOD_RES 14: note = Xaa=K or R
  MOD_RES 16: note = Xaa=K or T or Q
YINPYNDGTKYNEXFXG

SEQ ID NO: 260 - protein, 12 aa, synthetic construct
  MOD_RES 3: note = Xaa=M or V
  MOD_RES 4: note = Xaa=L or R
  MOD_RES 5: note = Xaa=T or R
  MOD_RES 6: note = Xaa=T or Y
  MOD_RES 7: note = Xaa=R or F
  MOD_RES 8: note = Xaa=S or inexistence
  MOD_RES 9: note = Xaa=L or inexistence
  MOD_RES 10: note = Xaa=F or inexistence
  MOD_RES 11: note = Xaa=A or T or V or L or D
GGXXXXXXXXXY

SEQ ID NO: 261 - protein, 11 aa, synthetic construct
  MOD_RES 5: note = Xaa=R or E or D
  MOD_RES 7: note = Xaa=G or S
  MOD_RES 8: note = Xaa=G or S
  MOD_RES 9: note = Xaa=Y or N
  MOD_RES 10: note = Xaa=L or F
  MOD_RES 11: note = Xaa=N or S
RASQXIXXXXX

SEQ ID NO: 262 - protein, 7 aa, synthetic construct
  MOD_RES 2: note = Xaa=A or T
  MOD_RES 4: note = Xaa=T or S
AXSXLDS

SEQ ID NO: 263 - protein, 9 aa, synthetic construct
  MOD_RES 5: note = Xaa=S or N
  MOD_RES 6: note = Xaa=Y or F
  MOD_RES 8: note = Xaa= P or Y
LQYAXXPXT

SEQ ID NO: 264 - protein, 11 aa, synthetic construct
  MOD_RES 2: note = Xaa=G or E
  MOD_RES 3: note = Xaa=G or A
  MOD_RES 4: note = Xaa=S or R
  MOD_RES 5: note = Xaa=S or A
  MOD_RES 6: note = Xaa=S or T
  MOD_RES 7: note = Xaa=Y or F
  MOD_RES 8: note = Xaa=V or inexistence
  MOD_RES 9: note = Xaa=V or inexistence
  MOD_RES 10: note = Xaa=M or inexistence
HXXXXXXXXDY

SEQ ID NO: 265 - protein, 17 aa, synthetic construct
  MOD_RES 16: note = Xaa=K or Q
  MOD_RES 17: note = Xaa=N or G
EFNPSNGRINYNEKFXX

SEQ ID NO: 266 - protein, 10 aa, synthetic construct
  MOD_RES 1: note = Xaa=S or R
XASSTVSYIH

SEQ ID NO: 267 - protein, 111 aa, synthetic construct
DIVLTQSPASLAVSPGQRATITCRASKSVSTSGYSYMHWYQKKPGQPPKLLIYLASNLESGVPARFSGSGSGTDFTLTINPVEAEDTANYYCQHSRELPWTFGQGTKVEIK

SEQ ID NO: 268 - protein, 122 aa, synthetic construct; identical to SEQ ID NO: 233

SEQ ID NO: 269 - DNA, 333 bp, synthetic construct
  source 1..333: mol_type = other DNA
gacatcgtgctgacacagagccctgcttctctggctgtgtctcctggccagagagccaccatcacctgtagagccagcaagagcgtgtccaccagcggctactcttacatgcactggtatcagaagaagcccggccagcctcctaagctgctgatctacctggctagcaacctcgaaagcggagtgcctgctagattttctggcagcggctctggcaccgacttcaccctgacaatcaaccccgtggaagccgaagacaccgccaactactactgccagcacagcagagagctgccctggacatttggccagggcaccaaggtggaaatcaag

SEQ ID NO: 270 - DNA, 366 bp, synthetic construct
  source 1..366: mol_type = other DNA
caggttcagctggtgcagtctggcagcgagctgaagaaacctggcgcctctgtgaaggtgtcctgcaaggctagcggctacatcttcaccaacttcggcatgaactgggtccgagaggctcctggacagggactcgaatggatgggctggatcaacacctacaccggcgagcagatctacgccgatggcttcacaggcagattcgtgttcagcctggacaccagcgtcagcacagcttacctgcagatcagctctctgaaggccgaggataccgccgtgtacttctgtgccagaggcgagatctactacggctacgacgtgggctttgtgtactggggccagggaacactggtcaccgttagctct

SEQ ID NO: 271 - DNA, 321 bp, synthetic construct
  source 1..321: mol_type = other DNA
gacatccagatgacacagagccctagcagcctgtctgccagcgtgggagacagagtgaccatcacctgtcaagccagccagaacgtgggcacaaacgtggcctggtatcagcagaagcctggccaggcccctaaggctctgatctacagcgccagctacttaaacagcggcgtgccctctagattcagcggctctggctctggcaccgacttcaccttcacaatctctagcctgcagcctgaggacatcgctacctacttctgccagcagtacaacagctacctgctgaccttcggctgcggcaccaaggtggaaatcaag

SEQ ID NO: 272 - DNA, 354 bp, synthetic construct
  source 1..354: mol_type = other DNA
caggttcagctggttcagtctggcgccgaagtgaagaaacctggcagcagcgtgaaggtgtcctgcaaggctagcggctacagcttcaccggctacaccatgaactgggtccgacaggctcctggacagtgcctcgaatggatgggcctgatcaacccttacaacggcggcaccagatacaaccagaaattccagggcagagtgaccattaccgcggacgagtctaccagcaccgcctacatggaactgagcagcctgagaagcgaggacaccgccgtgtactactgtgccagatgggctctgagatacggcatggactactggggccagggaaccctggttaccgttagctct

SEQ ID NO: 273 - protein, 14 aa, synthetic construct
GSTSGSGKSSEGKG

SEQ ID NO: 274 - protein, 7 aa, synthetic construct
GSGGGSG

SEQ ID NO: 275 - protein, 8 aa, synthetic construct
GGGSGGSG